European Patent Application EP 4 740 938 A1, published May 13, 2026. Title: KLK1融合蛋白的制备方法. Applicant: 礼邦医药(香港)有限公司. Application WO. The sequence listing filed with the application follows.

SEQUENCE LISTING (130 sequences)

SEQ ID NO: 1 - protein, 262 aa, synthetic construct
MWFLVLCLALSLGGTGAAPPIQSRIVGGWECEQHSQPWQAALYHFSTFQCGGILVHRQWVLTAAHCISDNYQLWLGRHNLFDDENTAQFVHVSESFPHPGFNMSLLENHTRQADEDYSHDLMLLRLTEPADTITDAVKVVELPTEEPEVGSTCLASGWGSIEPENFSFPDDLQCVDLKILPNDECKKAHVQKVTDFMLCVGHLEGGKDTCVGDSGGPLMCDGVLQGVTSWGYVPCGTPNKPSVAVRVLSYVKWIEDTIAENS

SEQ ID NO: 2 - protein, 238 aa, synthetic construct
IVGGWECEQHSQPWQAALYHFSTFQCGGILVHRQWVLTAAHCISDNYQLWLGRHNLFDDENTAQFVHVSESFPHPGFNMSLLENHTRQADEDYSHDLMLLRLTEPADTITDAVKVVELPTEEPEVGSTCLASGWGSIEPENFSFPDDLQCVDLKILPNDECKKAHVQKVTDFMLCVGHLEGGKDTCVGDSGGPLMCDGVLQGVTSWGYVPCGTPNKPSVAVRVLSYVKWIEDTIAENS

SEQ ID NO: 3 - protein, 261 aa, synthetic construct
MRFLILFLALSLGGIDAAPPVQSRIVGGFNCEKNSQPWQVAVYRFTKYQCGGILLNANWVLTAAHCHNDKYQVWLGKNNFLEDEPSAQHRLVSKAIPHPDFNMSLLNEHTPQPEDDYSNDLMLLRLKKPADITDVVKPIDLPTEEPKLGSTCLASGWGSITPVKYEYPDELQCVNLKLLPNEDCAKAHIEKVTDDMLCAGDMDGGKDTCAGDSGGPLICDGVLQGITSWGPSPCGKPNVPGIYTRVLNFNTWIRETMAEND

SEQ ID NO: 4 - protein, 5 aa, synthetic construct
DDDDK

SEQ ID NO: 5 - protein, 6 aa, synthetic construct
VDDDDK

SEQ ID NO: 6 - protein, 6 aa, synthetic construct
LVPRGS

SEQ ID NO: 7 - protein, 5 aa, synthetic construct
IEGRG

SEQ ID NO: 8 - protein, 7 aa, synthetic construct
ENLYFQG

SEQ ID NO: 9 - protein, 101 aa, synthetic construct
MSDQEAKPSTEDLGDKKEGEYIKLKVIGQDSSEIHFKVKMTTHLKKLKESYCQRQGVPMNSLRFLFEGQRIADNHTPKELGMEEEDVIEVYQEQTGGHSTV

SEQ ID NO: 10 - protein, 5 aa, synthetic construct
  VARIANT 3: note = X is any one of amino acid; note (original language) = X为任何氨基酸
LPXTG

SEQ ID NO: 11 - protein, 223 aa, synthetic construct
TCPPCPAPELLGGPSVFLFPPKPKDTLMISRTPEVTCVVVDVSHEDPEVKFNWYVDGVEVHNAKTKPREEQYNSTYRVVSVLTVLHQDWLNGKEYKCKVSNKALPAPIEKTISKAKGQPREPQVYTLPPSRDELTKNQVSLTCLVKGFYPSDIAVEWESNGQPENNYKTTPPVLDSDGSFFLYSKLTVDKSRWQQGNVFSCSVMHEALHNHYTQKSLSLSPGK

SEQ ID NO: 12 - protein, 225 aa, synthetic construct
GPPCPSCPAPEFLGGPSVFLFPPKPKDTLMISRTPEVTCVVVDVSQEDPEVQFNWYVDGVEVHNAKTKPREEQFNSTYRVVSVLTVLHQDWLNGKEYKCKVSNKGLPSSIEKTISKAKGQPREPQVYTLPPSQEEMTKNQVSLTCLVKGFYPSDIAVEWESNGQPENNYKTTPPVLDSDGSFFLYSRLTVDKSRWQEGNVFSCSVMHEALHNHYTQKSLSLSLGK

SEQ ID NO: 13 - protein, 223 aa, synthetic construct
TCPPCPAPELLGGPSVFLFPPKPKDTLYITREPEVTCVVVDVSHEDPEVKFNWYVDGVEVHNAKTKPREEQYNSTYRVVSVLTVLHQDWLNGKEYKCKVSNKALPAPIEKTISKAKGQPREPQVYTLPPSRDELTKNQVSLTCLVKGFYPSDIAVEWESNGQPENNYKTTPPVLDSDGSFFLYSKLTVDKSRWQQGNVFSCSVMHEALHNHYTQKSLSLSPGK

SEQ ID NO: 14 - protein, 225 aa, synthetic construct
GPPCPSCPAPEFLGGPSVFLFPPKPKDTLYITREPEVTCVVVDVSQEDPEVQFNWYVDGVEVHNAKTKPREEQFNSTYRVVSVLTVLHQDWLNGKEYKCKVSNKGLPSSIEKTISKAKGQPREPQVYTLPPSQEEMTKNQVSLTCLVKGFYPSDIAVEWESNGQPENNYKTTPPVLDSDGSFFLYSRLTVDKSRWQEGNVFSCSVMHEALHNHYTQKSLSLSLGK

SEQ ID NO: 15 - protein, 585 aa, synthetic construct [sequence omitted]

SEQ ID NO: 16 - protein, 6 aa, synthetic construct
HHHHHH

SEQ ID NO: 17 - protein, 4 aa, synthetic construct
GGGS

SEQ ID NO: 18 - protein, 5 aa, synthetic construct
GGGGS

SEQ ID NO: 19 - protein, 6 aa, synthetic construct
GGGGGS

SEQ ID NO: 20 - protein, 10 aa, synthetic construct
GGGGSGGGGS

SEQ ID NO: 21 - protein, 7 aa, synthetic construct
GGGSSSS

SEQ ID NO: 22 - protein, 7 aa, synthetic construct
GSSGSSG

SEQ ID NO: 23 - protein, 5 aa, synthetic construct
EAAAK

SEQ ID NO: 24 - protein, 18 aa, synthetic construct
MWFLVLCLALSLGGTGAA

SEQ ID NO: 25 - protein, 20 aa, synthetic construct
MYRMQLLSCIALSLALVTNS

SEQ ID NO: 26 - protein, 493 aa, synthetic construct
MWFLVLCLALSLGGTGAAGGHHHHHHVDDDDKIVGGWECEQHSQPWQAALYHFSTFQCGGILVHRQWVLTAAHCISDNYQLWLGRHNLFDDENTAQFVHVSESFPHPGFNMSLLENHTRQADEDYSHDLMLLRLTEPADTITDAVKVVELPTEEPEVGSTCLASGWGSIEPENFSFPDDLQCVDLKILPNDECKKAHVQKVTDFMLCVGHLEGGKDTCVGDSGGPLMCDGVLQGVTSWGYVPCGTPNKPSVAVRVLSYVKWIEDTIAENSTCPPCPAPELLGGPSVFLFPPKPKDTLMISRTPEVTCVVVDVSHEDPEVKFNWYVDGVEVHNAKTKPREEQYNSTYRVVSVLTVLHQDWLNGKEYKCKVSNKALPAPIEKTISKAKGQPREPQVYTLPPSRDELTKNQVSLTCLVKGFYPSDIAVEWESNGQPENNYKTTPPVLDSDGSFFLYSKLTVDKSRWQQGNVFSCSVMHEALHNHYTQKSLSLSPGK

SEQ ID NO: 27 - protein, 500 aa, synthetic construct
MWFLVLCLALSLGGTGAAGGHHHHHHVDDDDKIVGGWECEQHSQPWQAALYHFSTFQCGGILVHRQWVLTAAHCISDNYQLWLGRHNLFDDENTAQFVHVSESFPHPGFNMSLLENHTRQADEDYSHDLMLLRLTEPADTITDAVKVVELPTEEPEVGSTCLASGWGSIEPENFSFPDDLQCVDLKILPNDECKKAHVQKVTDFMLCVGHLEGGKDTCVGDSGGPLMCDGVLQGVTSWGYVPCGTPNKPSVAVRVLSYVKWIEDTIAENSGGGSSSSTCPPCPAPELLGGPSVFLFPPKPKDTLMISRTPEVTCVVVDVSHEDPEVKFNWYVDGVEVHNAKTKPREEQYNSTYRVVSVLTVLHQDWLNGKEYKCKVSNKALPAPIEKTISKAKGQPREPQVYTLPPSRDELTKNQVSLTCLVKGFYPSDIAVEWESNGQPENNYKTTPPVLDSDGSFFLYSKLTVDKSRWQQGNVFSCSVMHEALHNHYTQKSLSLSPGK

SEQ ID NO: 28 - protein, 498 aa, synthetic construct
MWFLVLCLALSLGGTGAAGGHHHHHHVDDDDKIVGGWECEQHSQPWQAALYHFSTFQCGGILVHRQWVLTAAHCISDNYQLWLGRHNLFDDENTAQFVHVSESFPHPGFNMSLLENHTRQADEDYSHDLMLLRLTEPADTITDAVKVVELPTEEPEVGSTCLASGWGSIEPENFSFPDDLQCVDLKILPNDECKKAHVQKVTDFMLCVGHLEGGKDTCVGDSGGPLMCDGVLQGVTSWGYVPCGTPNKPSVAVRVLSYVKWIEDTIAENSEAAAKTCPPCPAPELLGGPSVFLFPPKPKDTLMISRTPEVTCVVVDVSHEDPEVKFNWYVDGVEVHNAKTKPREEQYNSTYRVVSVLTVLHQDWLNGKEYKCKVSNKALPAPIEKTISKAKGQPREPQVYTLPPSRDELTKNQVSLTCLVKGFYPSDIAVEWESNGQPENNYKTTPPVLDSDGSFFLYSKLTVDKSRWQQGNVFSCSVMHEALHNHYTQKSLSLSPGK

SEQ ID NO: 29 - protein, 502 aa, synthetic construct
MYRMQLLSCIALSLALVTNSGGHHHHHHVDDDDKIVGGWECEQHSQPWQAALYHFSTFQCGGILVHRQWVLTAAHCISDNYQLWLGRHNLFDDENTAQFVHVSESFPHPGFNMSLLENHTRQADEDYSHDLMLLRLTEPADTITDAVKVVELPTEEPEVGSTCLASGWGSIEPENFSFPDDLQCVDLKILPNDECKKAHVQKVTDFMLCVGHLEGGKDTCVGDSGGPLMCDGVLQGVTSWGYVPCGTPNKPSVAVRVLSYVKWIEDTIAENSGGGSSSSTCPPCPAPELLGGPSVFLFPPKPKDTLMISRTPEVTCVVVDVSHEDPEVKFNWYVDGVEVHNAKTKPREEQYNSTYRVVSVLTVLHQDWLNGKEYKCKVSNKALPAPIEKTISKAKGQPREPQVYTLPPSRDELTKNQVSLTCLVKGFYPSDIAVEWESNGQPENNYKTTPPVLDSDGSFFLYSKLTVDKSRWQQGNVFSCSVMHEALHNHYTQKSLSLSPGK

SEQ ID NO: 30 - protein, 500 aa, synthetic construct
MYRMQLLSCIALSLALVTNSGGHHHHHHVDDDDKIVGGWECEQHSQPWQAALYHFSTFQCGGILVHRQWVLTAAHCISDNYQLWLGRHNLFDDENTAQFVHVSESFPHPGFNMSLLENHTRQADEDYSHDLMLLRLTEPADTITDAVKVVELPTEEPEVGSTCLASGWGSIEPENFSFPDDLQCVDLKILPNDECKKAHVQKVTDFMLCVGHLEGGKDTCVGDSGGPLMCDGVLQGVTSWGYVPCGTPNKPSVAVRVLSYVKWIEDTIAENSEAAAKTCPPCPAPELLGGPSVFLFPPKPKDTLMISRTPEVTCVVVDVSHEDPEVKFNWYVDGVEVHNAKTKPREEQYNSTYRVVSVLTVLHQDWLNGKEYKCKVSNKALPAPIEKTISKAKGQPREPQVYTLPPSRDELTKNQVSLTCLVKGFYPSDIAVEWESNGQPENNYKTTPPVLDSDGSFFLYSKLTVDKSRWQQGNVFSCSVMHEALHNHYTQKSLSLSPGK

SEQ ID NO: 31 - protein, 500 aa, synthetic construct
MWFLVLCLALSLGGTGAAGGHHHHHHVDDDDKIVGGWECEQHSQPWQAALYHFSTFQCGGILVHRQWVLTAAHCISDNYQLWLGRHNLFDDENTAQFVHVSESFPHPGFNMSLLENHTRQADEDYSHDLMLLRLTEPADTITDAVKVVELPTEEPEVGSTCLASGWGSIEPENFSFPDDLQCVDLKILPNDECKKAHVQKVTDFMLCVGHLEGGKDTCVGDSGGPLMCDGVLQGVTSWGYVPCGTPNKPSVAVRVLSYVKWIEDTIAENSGSSGSSGTCPPCPAPELLGGPSVFLFPPKPKDTLMISRTPEVTCVVVDVSHEDPEVKFNWYVDGVEVHNAKTKPREEQYNSTYRVVSVLTVLHQDWLNGKEYKCKVSNKALPAPIEKTISKAKGQPREPQVYTLPPSRDELTKNQVSLTCLVKGFYPSDIAVEWESNGQPENNYKTTPPVLDSDGSFFLYSKLTVDKSRWQQGNVFSCSVMHEALHNHYTQKSLSLSPGK

SEQ ID NO: 32 - protein, 500 aa, synthetic construct
MWFLVLCLALSLGGTGAAGGHHHHHHVDDDDKIVGGWECEQHSQPWQAALYHFSTFQCGGILVHRQWVLTAAHCISDNYQLWLGRHNLFDDENTAQFVHVSESFPHPGFNMSLLENHTRQADEDYSHDLMLLRLTEPADTITDAVKVVELPTEEPEVGSTCLASGWGSIEPENFSFPDDLQCVDLKILPNDECKKAHVQKVTDFMLCVGHLEGGKDTCVGDSGGPLMCDGVLQGVTSWGYVPCGTPNKPSVAVRVLSYVKWIEDTIAENSGSSGSSGTCPPCPAPELLGGPSVFLFPPKPKDTLYITREPEVTCVVVDVSHEDPEVKFNWYVDGVEVHNAKTKPREEQYNSTYRVVSVLTVLHQDWLNGKEYKCKVSNKALPAPIEKTISKAKGQPREPQVYTLPPSRDELTKNQVSLTCLVKGFYPSDIAVEWESNGQPENNYKTTPPVLDSDGSFFLYSKLTVDKSRWQQGNVFSCSVMHEALHNHYTQKSLSLSPGK

SEQ ID NO: 33 - protein, 502 aa, synthetic construct
MWFLVLCLALSLGGTGAAGGHHHHHHVDDDDKIVGGWECEQHSQPWQAALYHFSTFQCGGILVHRQWVLTAAHCISDNYQLWLGRHNLFDDENTAQFVHVSESFPHPGFNMSLLENHTRQADEDYSHDLMLLRLTEPADTITDAVKVVELPTEEPEVGSTCLASGWGSIEPENFSFPDDLQCVDLKILPNDECKKAHVQKVTDFMLCVGHLEGGKDTCVGDSGGPLMCDGVLQGVTSWGYVPCGTPNKPSVAVRVLSYVKWIEDTIAENSGSSGSSGGPPCPSCPAPEFLGGPSVFLFPPKPKDTLMISRTPEVTCVVVDVSQEDPEVQFNWYVDGVEVHNAKTKPREEQFNSTYRVVSVLTVLHQDWLNGKEYKCKVSNKGLPSSIEKTISKAKGQPREPQVYTLPPSQEEMTKNQVSLTCLVKGFYPSDIAVEWESNGQPENNYKTTPPVLDSDGSFFLYSRLTVDKSRWQEGNVFSCSVMHEALHNHYTQKSLSLSLGK

SEQ ID NO: 34 - protein, 502 aa, synthetic construct
MWFLVLCLALSLGGTGAAGGHHHHHHVDDDDKIVGGWECEQHSQPWQAALYHFSTFQCGGILVHRQWVLTAAHCISDNYQLWLGRHNLFDDENTAQFVHVSESFPHPGFNMSLLENHTRQADEDYSHDLMLLRLTEPADTITDAVKVVELPTEEPEVGSTCLASGWGSIEPENFSFPDDLQCVDLKILPNDECKKAHVQKVTDFMLCVGHLEGGKDTCVGDSGGPLMCDGVLQGVTSWGYVPCGTPNKPSVAVRVLSYVKWIEDTIAENSGSSGSSGGPPCPSCPAPEFLGGPSVFLFPPKPKDTLYITREPEVTCVVVDVSQEDPEVQFNWYVDGVEVHNAKTKPREEQFNSTYRVVSVLTVLHQDWLNGKEYKCKVSNKGLPSSIEKTISKAKGQPREPQVYTLPPSQEEMTKNQVSLTCLVKGFYPSDIAVEWESNGQPENNYKTTPPVLDSDGSFFLYSRLTVDKSRWQEGNVFSCSVMHEALHNHYTQKSLSLSLGK

SEQ ID NO: 35 - protein, 503 aa, synthetic construct
MWFLVLCLALSLGGTGAAGGHHHHHHVDDDDKIVGGWECEQHSQPWQAALYHFSTFQCGGILVHRQWVLTAAHCISDNYQLWLGRHNLFDDENTAQFVHVSESFPHPGFNMSLLENHTRQADEDYSHDLMLLRLTEPADTITDAVKVVELPTEEPEVGSTCLASGWGSIEPENFSFPDDLQCVDLKILPNDECKKAHVQKVTDFMLCVGHLEGGKDTCVGDSGGPLMCDGVLQGVTSWGYVPCGTPNKPSVAVRVLSYVKWIEDTIAENSGGGGSGGGGSTCPPCPAPELLGGPSVFLFPPKPKDTLMISRTPEVTCVVVDVSHEDPEVKFNWYVDGVEVHNAKTKPREEQYNSTYRVVSVLTVLHQDWLNGKEYKCKVSNKALPAPIEKTISKAKGQPREPQVYTLPPSRDELTKNQVSLTCLVKGFYPSDIAVEWESNGQPENNYKTTPPVLDSDGSFFLYSKLTVDKSRWQQGNVFSCSVMHEALHNHYTQKSLSLSPGK

SEQ ID NO: 36 - protein, 473 aa, synthetic construct
HHHHHHVDDDDKIVGGWECEQHSQPWQAALYHFSTFQCGGILVHRQWVLTAAHCISDNYQLWLGRHNLFDDENTAQFVHVSESFPHPGFNMSLLENHTRQADEDYSHDLMLLRLTEPADTITDAVKVVELPTEEPEVGSTCLASGWGSIEPENFSFPDDLQCVDLKILPNDECKKAHVQKVTDFMLCVGHLEGGKDTCVGDSGGPLMCDGVLQGVTSWGYVPCGTPNKPSVAVRVLSYVKWIEDTIAENSTCPPCPAPELLGGPSVFLFPPKPKDTLMISRTPEVTCVVVDVSHEDPEVKFNWYVDGVEVHNAKTKPREEQYNSTYRVVSVLTVLHQDWLNGKEYKCKVSNKALPAPIEKTISKAKGQPREPQVYTLPPSRDELTKNQVSLTCLVKGFYPSDIAVEWESNGQPENNYKTTPPVLDSDGSFFLYSKLTVDKSRWQQGNVFSCSVMHEALHNHYTQKSLSLSPGK

SEQ ID NO: 37 - protein, 480 aa, synthetic construct
HHHHHHVDDDDKIVGGWECEQHSQPWQAALYHFSTFQCGGILVHRQWVLTAAHCISDNYQLWLGRHNLFDDENTAQFVHVSESFPHPGFNMSLLENHTRQADEDYSHDLMLLRLTEPADTITDAVKVVELPTEEPEVGSTCLASGWGSIEPENFSFPDDLQCVDLKILPNDECKKAHVQKVTDFMLCVGHLEGGKDTCVGDSGGPLMCDGVLQGVTSWGYVPCGTPNKPSVAVRVLSYVKWIEDTIAENSGGGSSSSTCPPCPAPELLGGPSVFLFPPKPKDTLMISRTPEVTCVVVDVSHEDPEVKFNWYVDGVEVHNAKTKPREEQYNSTYRVVSVLTVLHQDWLNGKEYKCKVSNKALPAPIEKTISKAKGQPREPQVYTLPPSRDELTKNQVSLTCLVKGFYPSDIAVEWESNGQPENNYKTTPPVLDSDGSFFLYSKLTVDKSRWQQGNVFSCSVMHEALHNHYTQKSLSLSPGK

SEQ ID NO: 38 - protein, 478 aa, synthetic construct
HHHHHHVDDDDKIVGGWECEQHSQPWQAALYHFSTFQCGGILVHRQWVLTAAHCISDNYQLWLGRHNLFDDENTAQFVHVSESFPHPGFNMSLLENHTRQADEDYSHDLMLLRLTEPADTITDAVKVVELPTEEPEVGSTCLASGWGSIEPENFSFPDDLQCVDLKILPNDECKKAHVQKVTDFMLCVGHLEGGKDTCVGDSGGPLMCDGVLQGVTSWGYVPCGTPNKPSVAVRVLSYVKWIEDTIAENSEAAAKTCPPCPAPELLGGPSVFLFPPKPKDTLMISRTPEVTCVVVDVSHEDPEVKFNWYVDGVEVHNAKTKPREEQYNSTYRVVSVLTVLHQDWLNGKEYKCKVSNKALPAPIEKTISKAKGQPREPQVYTLPPSRDELTKNQVSLTCLVKGFYPSDIAVEWESNGQPENNYKTTPPVLDSDGSFFLYSKLTVDKSRWQQGNVFSCSVMHEALHNHYTQKSLSLSPGK

SEQ ID NO: 39 - protein, 480 aa, synthetic construct; identical to SEQ ID NO: 37

SEQ ID NO: 40 - protein, 478 aa, synthetic construct; identical to SEQ ID NO: 38

SEQ ID NO: 41 - protein, 480 aa, synthetic construct
HHHHHHVDDDDKIVGGWECEQHSQPWQAALYHFSTFQCGGILVHRQWVLTAAHCISDNYQLWLGRHNLFDDENTAQFVHVSESFPHPGFNMSLLENHTRQADEDYSHDLMLLRLTEPADTITDAVKVVELPTEEPEVGSTCLASGWGSIEPENFSFPDDLQCVDLKILPNDECKKAHVQKVTDFMLCVGHLEGGKDTCVGDSGGPLMCDGVLQGVTSWGYVPCGTPNKPSVAVRVLSYVKWIEDTIAENSGSSGSSGTCPPCPAPELLGGPSVFLFPPKPKDTLMISRTPEVTCVVVDVSHEDPEVKFNWYVDGVEVHNAKTKPREEQYNSTYRVVSVLTVLHQDWLNGKEYKCKVSNKALPAPIEKTISKAKGQPREPQVYTLPPSRDELTKNQVSLTCLVKGFYPSDIAVEWESNGQPENNYKTTPPVLDSDGSFFLYSKLTVDKSRWQQGNVFSCSVMHEALHNHYTQKSLSLSPGK

SEQ ID NO: 42 - protein, 480 aa, synthetic construct
HHHHHHVDDDDKIVGGWECEQHSQPWQAALYHFSTFQCGGILVHRQWVLTAAHCISDNYQLWLGRHNLFDDENTAQFVHVSESFPHPGFNMSLLENHTRQADEDYSHDLMLLRLTEPADTITDAVKVVELPTEEPEVGSTCLASGWGSIEPENFSFPDDLQCVDLKILPNDECKKAHVQKVTDFMLCVGHLEGGKDTCVGDSGGPLMCDGVLQGVTSWGYVPCGTPNKPSVAVRVLSYVKWIEDTIAENSGSSGSSGTCPPCPAPELLGGPSVFLFPPKPKDTLYITREPEVTCVVVDVSHEDPEVKFNWYVDGVEVHNAKTKPREEQYNSTYRVVSVLTVLHQDWLNGKEYKCKVSNKALPAPIEKTISKAKGQPREPQVYTLPPSRDELTKNQVSLTCLVKGFYPSDIAVEWESNGQPENNYKTTPPVLDSDGSFFLYSKLTVDKSRWQQGNVFSCSVMHEALHNHYTQKSLSLSPGK

SEQ ID NO: 43 - protein, 482 aa, synthetic construct
HHHHHHVDDDDKIVGGWECEQHSQPWQAALYHFSTFQCGGILVHRQWVLTAAHCISDNYQLWLGRHNLFDDENTAQFVHVSESFPHPGFNMSLLENHTRQADEDYSHDLMLLRLTEPADTITDAVKVVELPTEEPEVGSTCLASGWGSIEPENFSFPDDLQCVDLKILPNDECKKAHVQKVTDFMLCVGHLEGGKDTCVGDSGGPLMCDGVLQGVTSWGYVPCGTPNKPSVAVRVLSYVKWIEDTIAENSGSSGSSGGPPCPSCPAPEFLGGPSVFLFPPKPKDTLMISRTPEVTCVVVDVSQEDPEVQFNWYVDGVEVHNAKTKPREEQFNSTYRVVSVLTVLHQDWLNGKEYKCKVSNKGLPSSIEKTISKAKGQPREPQVYTLPPSQEEMTKNQVSLTCLVKGFYPSDIAVEWESNGQPENNYKTTPPVLDSDGSFFLYSRLTVDKSRWQEGNVFSCSVMHEALHNHYTQKSLSLSLGK

SEQ ID NO: 44 - protein, 482 aa, synthetic construct
HHHHHHVDDDDKIVGGWECEQHSQPWQAALYHFSTFQCGGILVHRQWVLTAAHCISDNYQLWLGRHNLFDDENTAQFVHVSESFPHPGFNMSLLENHTRQADEDYSHDLMLLRLTEPADTITDAVKVVELPTEEPEVGSTCLASGWGSIEPENFSFPDDLQCVDLKILPNDECKKAHVQKVTDFMLCVGHLEGGKDTCVGDSGGPLMCDGVLQGVTSWGYVPCGTPNKPSVAVRVLSYVKWIEDTIAENSGSSGSSGGPPCPSCPAPEFLGGPSVFLFPPKPKDTLYITREPEVTCVVVDVSQEDPEVQFNWYVDGVEVHNAKTKPREEQFNSTYRVVSVLTVLHQDWLNGKEYKCKVSNKGLPSSIEKTISKAKGQPREPQVYTLPPSQEEMTKNQVSLTCLVKGFYPSDIAVEWESNGQPENNYKTTPPVLDSDGSFFLYSRLTVDKSRWQEGNVFSCSVMHEALHNHYTQKSLSLSLGK

SEQ ID NO: 45 - protein, 483 aa, synthetic construct
HHHHHHVDDDDKIVGGWECEQHSQPWQAALYHFSTFQCGGILVHRQWVLTAAHCISDNYQLWLGRHNLFDDENTAQFVHVSESFPHPGFNMSLLENHTRQADEDYSHDLMLLRLTEPADTITDAVKVVELPTEEPEVGSTCLASGWGSIEPENFSFPDDLQCVDLKILPNDECKKAHVQKVTDFMLCVGHLEGGKDTCVGDSGGPLMCDGVLQGVTSWGYVPCGTPNKPSVAVRVLSYVKWIEDTIAENSGGGGSGGGGSTCPPCPAPELLGGPSVFLFPPKPKDTLMISRTPEVTCVVVDVSHEDPEVKFNWYVDGVEVHNAKTKPREEQYNSTYRVVSVLTVLHQDWLNGKEYKCKVSNKALPAPIEKTISKAKGQPREPQVYTLPPSRDELTKNQVSLTCLVKGFYPSDIAVEWESNGQPENNYKTTPPVLDSDGSFFLYSKLTVDKSRWQQGNVFSCSVMHEALHNHYTQKSLSLSPGK

SEQ ID NO: 46 - protein, 467 aa, synthetic construct
VDDDDKIVGGWECEQHSQPWQAALYHFSTFQCGGILVHRQWVLTAAHCISDNYQLWLGRHNLFDDENTAQFVHVSESFPHPGFNMSLLENHTRQADEDYSHDLMLLRLTEPADTITDAVKVVELPTEEPEVGSTCLASGWGSIEPENFSFPDDLQCVDLKILPNDECKKAHVQKVTDFMLCVGHLEGGKDTCVGDSGGPLMCDGVLQGVTSWGYVPCGTPNKPSVAVRVLSYVKWIEDTIAENSTCPPCPAPELLGGPSVFLFPPKPKDTLMISRTPEVTCVVVDVSHEDPEVKFNWYVDGVEVHNAKTKPREEQYNSTYRVVSVLTVLHQDWLNGKEYKCKVSNKALPAPIEKTISKAKGQPREPQVYTLPPSRDELTKNQVSLTCLVKGFYPSDIAVEWESNGQPENNYKTTPPVLDSDGSFFLYSKLTVDKSRWQQGNVFSCSVMHEALHNHYTQKSLSLSPGK

SEQ ID NO: 47 - protein, 474 aa, synthetic construct
VDDDDKIVGGWECEQHSQPWQAALYHFSTFQCGGILVHRQWVLTAAHCISDNYQLWLGRHNLFDDENTAQFVHVSESFPHPGFNMSLLENHTRQADEDYSHDLMLLRLTEPADTITDAVKVVELPTEEPEVGSTCLASGWGSIEPENFSFPDDLQCVDLKILPNDECKKAHVQKVTDFMLCVGHLEGGKDTCVGDSGGPLMCDGVLQGVTSWGYVPCGTPNKPSVAVRVLSYVKWIEDTIAENSGGGSSSSTCPPCPAPELLGGPSVFLFPPKPKDTLMISRTPEVTCVVVDVSHEDPEVKFNWYVDGVEVHNAKTKPREEQYNSTYRVVSVLTVLHQDWLNGKEYKCKVSNKALPAPIEKTISKAKGQPREPQVYTLPPSRDELTKNQVSLTCLVKGFYPSDIAVEWESNGQPENNYKTTPPVLDSDGSFFLYSKLTVDKSRWQQGNVFSCSVMHEALHNHYTQKSLSLSPGK

SEQ ID NO: 48 - protein, 472 aa, synthetic construct
VDDDDKIVGGWECEQHSQPWQAALYHFSTFQCGGILVHRQWVLTAAHCISDNYQLWLGRHNLFDDENTAQFVHVSESFPHPGFNMSLLENHTRQADEDYSHDLMLLRLTEPADTITDAVKVVELPTEEPEVGSTCLASGWGSIEPENFSFPDDLQCVDLKILPNDECKKAHVQKVTDFMLCVGHLEGGKDTCVGDSGGPLMCDGVLQGVTSWGYVPCGTPNKPSVAVRVLSYVKWIEDTIAENSEAAAKTCPPCPAPELLGGPSVFLFPPKPKDTLMISRTPEVTCVVVDVSHEDPEVKFNWYVDGVEVHNAKTKPREEQYNSTYRVVSVLTVLHQDWLNGKEYKCKVSNKALPAPIEKTISKAKGQPREPQVYTLPPSRDELTKNQVSLTCLVKGFYPSDIAVEWESNGQPENNYKTTPPVLDSDGSFFLYSKLTVDKSRWQQGNVFSCSVMHEALHNHYTQKSLSLSPGK

SEQ ID NO: 49 - protein, 474 aa, synthetic construct; identical to SEQ ID NO: 47

SEQ ID NO: 50 - protein, 472 aa, synthetic construct; identical to SEQ ID NO: 48

SEQ ID NO: 51 - protein, 474 aa, synthetic construct
VDDDDKIVGGWECEQHSQPWQAALYHFSTFQCGGILVHRQWVLTAAHCISDNYQLWLGRHNLFDDENTAQFVHVSESFPHPGFNMSLLENHTRQADEDYSHDLMLLRLTEPADTITDAVKVVELPTEEPEVGSTCLASGWGSIEPENFSFPDDLQCVDLKILPNDECKKAHVQKVTDFMLCVGHLEGGKDTCVGDSGGPLMCDGVLQGVTSWGYVPCGTPNKPSVAVRVLSYVKWIEDTIAENSGSSGSSGTCPPCPAPELLGGPSVFLFPPKPKDTLMISRTPEVTCVVVDVSHEDPEVKFNWYVDGVEVHNAKTKPREEQYNSTYRVVSVLTVLHQDWLNGKEYKCKVSNKALPAPIEKTISKAKGQPREPQVYTLPPSRDELTKNQVSLTCLVKGFYPSDIAVEWESNGQPENNYKTTPPVLDSDGSFFLYSKLTVDKSRWQQGNVFSCSVMHEALHNHYTQKSLSLSPGK

SEQ ID NO: 52 - protein, 474 aa, synthetic construct
VDDDDKIVGGWECEQHSQPWQAALYHFSTFQCGGILVHRQWVLTAAHCISDNYQLWLGRHNLFDDENTAQFVHVSESFPHPGFNMSLLENHTRQADEDYSHDLMLLRLTEPADTITDAVKVVELPTEEPEVGSTCLASGWGSIEPENFSFPDDLQCVDLKILPNDECKKAHVQKVTDFMLCVGHLEGGKDTCVGDSGGPLMCDGVLQGVTSWGYVPCGTPNKPSVAVRVLSYVKWIEDTIAENSGSSGSSGTCPPCPAPELLGGPSVFLFPPKPKDTLYITREPEVTCVVVDVSHEDPEVKFNWYVDGVEVHNAKTKPREEQYNSTYRVVSVLTVLHQDWLNGKEYKCKVSNKALPAPIEKTISKAKGQPREPQVYTLPPSRDELTKNQVSLTCLVKGFYPSDIAVEWESNGQPENNYKTTPPVLDSDGSFFLYSKLTVDKSRWQQGNVFSCSVMHEALHNHYTQKSLSLSPGK

SEQ ID NO: 53 - protein, 476 aa, synthetic construct
VDDDDKIVGGWECEQHSQPWQAALYHFSTFQCGGILVHRQWVLTAAHCISDNYQLWLGRHNLFDDENTAQFVHVSESFPHPGFNMSLLENHTRQADEDYSHDLMLLRLTEPADTITDAVKVVELPTEEPEVGSTCLASGWGSIEPENFSFPDDLQCVDLKILPNDECKKAHVQKVTDFMLCVGHLEGGKDTCVGDSGGPLMCDGVLQGVTSWGYVPCGTPNKPSVAVRVLSYVKWIEDTIAENSGSSGSSGGPPCPSCPAPEFLGGPSVFLFPPKPKDTLMISRTPEVTCVVVDVSQEDPEVQFNWYVDGVEVHNAKTKPREEQFNSTYRVVSVLTVLHQDWLNGKEYKCKVSNKGLPSSIEKTISKAKGQPREPQVYTLPPSQEEMTKNQVSLTCLVKGFYPSDIAVEWESNGQPENNYKTTPPVLDSDGSFFLYSRLTVDKSRWQEGNVFSCSVMHEALHNHYTQKSLSLSLGK

SEQ ID NO: 54 - protein, 476 aa, synthetic construct
VDDDDKIVGGWECEQHSQPWQAALYHFSTFQCGGILVHRQWVLTAAHCISDNYQLWLGRHNLFDDENTAQFVHVSESFPHPGFNMSLLENHTRQADEDYSHDLMLLRLTEPADTITDAVKVVELPTEEPEVGSTCLASGWGSIEPENFSFPDDLQCVDLKILPNDECKKAHVQKVTDFMLCVGHLEGGKDTCVGDSGGPLMCDGVLQGVTSWGYVPCGTPNKPSVAVRVLSYVKWIEDTIAENSGSSGSSGGPPCPSCPAPEFLGGPSVFLFPPKPKDTLYITREPEVTCVVVDVSQEDPEVQFNWYVDGVEVHNAKTKPREEQFNSTYRVVSVLTVLHQDWLNGKEYKCKVSNKGLPSSIEKTISKAKGQPREPQVYTLPPSQEEMTKNQVSLTCLVKGFYPSDIAVEWESNGQPENNYKTTPPVLDSDGSFFLYSRLTVDKSRWQEGNVFSCSVMHEALHNHYTQKSLSLSLGK

SEQ ID NO: 55 - protein, 477 aa, synthetic construct
VDDDDKIVGGWECEQHSQPWQAALYHFSTFQCGGILVHRQWVLTAAHCISDNYQLWLGRHNLFDDENTAQFVHVSESFPHPGFNMSLLENHTRQADEDYSHDLMLLRLTEPADTITDAVKVVELPTEEPEVGSTCLASGWGSIEPENFSFPDDLQCVDLKILPNDECKKAHVQKVTDFMLCVGHLEGGKDTCVGDSGGPLMCDGVLQGVTSWGYVPCGTPNKPSVAVRVLSYVKWIEDTIAENSGGGGSGGGGSTCPPCPAPELLGGPSVFLFPPKPKDTLMISRTPEVTCVVVDVSHEDPEVKFNWYVDGVEVHNAKTKPREEQYNSTYRVVSVLTVLHQDWLNGKEYKCKVSNKALPAPIEKTISKAKGQPREPQVYTLPPSRDELTKNQVSLTCLVKGFYPSDIAVEWESNGQPENNYKTTPPVLDSDGSFFLYSKLTVDKSRWQQGNVFSCSVMHEALHNHYTQKSLSLSPGK

SEQ ID NO: 56 - protein, 461 aa, synthetic construct
IVGGWECEQHSQPWQAALYHFSTFQCGGILVHRQWVLTAAHCISDNYQLWLGRHNLFDDENTAQFVHVSESFPHPGFNMSLLENHTRQADEDYSHDLMLLRLTEPADTITDAVKVVELPTEEPEVGSTCLASGWGSIEPENFSFPDDLQCVDLKILPNDECKKAHVQKVTDFMLCVGHLEGGKDTCVGDSGGPLMCDGVLQGVTSWGYVPCGTPNKPSVAVRVLSYVKWIEDTIAENSTCPPCPAPELLGGPSVFLFPPKPKDTLMISRTPEVTCVVVDVSHEDPEVKFNWYVDGVEVHNAKTKPREEQYNSTYRVVSVLTVLHQDWLNGKEYKCKVSNKALPAPIEKTISKAKGQPREPQVYTLPPSRDELTKNQVSLTCLVKGFYPSDIAVEWESNGQPENNYKTTPPVLDSDGSFFLYSKLTVDKSRWQQGNVFSCSVMHEALHNHYTQKSLSLSPGK

SEQ ID NO: 57 - protein, 468 aa, synthetic construct
IVGGWECEQHSQPWQAALYHFSTFQCGGILVHRQWVLTAAHCISDNYQLWLGRHNLFDDENTAQFVHVSESFPHPGFNMSLLENHTRQADEDYSHDLMLLRLTEPADTITDAVKVVELPTEEPEVGSTCLASGWGSIEPENFSFPDDLQCVDLKILPNDECKKAHVQKVTDFMLCVGHLEGGKDTCVGDSGGPLMCDGVLQGVTSWGYVPCGTPNKPSVAVRVLSYVKWIEDTIAENSGGGSSSSTCPPCPAPELLGGPSVFLFPPKPKDTLMISRTPEVTCVVVDVSHEDPEVKFNWYVDGVEVHNAKTKPREEQYNSTYRVVSVLTVLHQDWLNGKEYKCKVSNKALPAPIEKTISKAKGQPREPQVYTLPPSRDELTKNQVSLTCLVKGFYPSDIAVEWESNGQPENNYKTTPPVLDSDGSFFLYSKLTVDKSRWQQGNVFSCSVMHEALHNHYTQKSLSLSPGK

SEQ ID NO: 58 - protein, 466 aa, synthetic construct
IVGGWECEQHSQPWQAALYHFSTFQCGGILVHRQWVLTAAHCISDNYQLWLGRHNLFDDENTAQFVHVSESFPHPGFNMSLLENHTRQADEDYSHDLMLLRLTEPADTITDAVKVVELPTEEPEVGSTCLASGWGSIEPENFSFPDDLQCVDLKILPNDECKKAHVQKVTDFMLCVGHLEGGKDTCVGDSGGPLMCDGVLQGVTSWGYVPCGTPNKPSVAVRVLSYVKWIEDTIAENSEAAAKTCPPCPAPELLGGPSVFLFPPKPKDTLMISRTPEVTCVVVDVSHEDPEVKFNWYVDGVEVHNAKTKPREEQYNSTYRVVSVLTVLHQDWLNGKEYKCKVSNKALPAPIEKTISKAKGQPREPQVYTLPPSRDELTKNQVSLTCLVKGFYPSDIAVEWESNGQPENNYKTTPPVLDSDGSFFLYSKLTVDKSRWQQGNVFSCSVMHEALHNHYTQKSLSLSPGK

SEQ ID NO: 59 - protein, 468 aa, synthetic construct; identical to SEQ ID NO: 57

SEQ ID NO: 60 - protein, 466 aa, synthetic construct; identical to SEQ ID NO: 58

SEQ ID NO: 61 - protein, 468 aa, synthetic construct
IVGGWECEQHSQPWQAALYHFSTFQCGGILVHRQWVLTAAHCISDNYQLWLGRHNLFDDENTAQFVHVSESFPHPGFNMSLLENHTRQADEDYSHDLMLLRLTEPADTITDAVKVVELPTEEPEVGSTCLASGWGSIEPENFSFPDDLQCVDLKILPNDECKKAHVQKVTDFMLCVGHLEGGKDTCVGDSGGPLMCDGVLQGVTSWGYVPCGTPNKPSVAVRVLSYVKWIEDTIAENSGSSGSSGTCPPCPAPELLGGPSVFLFPPKPKDTLMISRTPEVTCVVVDVSHEDPEVKFNWYVDGVEVHNAKTKPREEQYNSTYRVVSVLTVLHQDWLNGKEYKCKVSNKALPAPIEKTISKAKGQPREPQVYTLPPSRDELTKNQVSLTCLVKGFYPSDIAVEWESNGQPENNYKTTPPVLDSDGSFFLYSKLTVDKSRWQQGNVFSCSVMHEALHNHYTQKSLSLSPGK

SEQ ID NO: 62 - protein, 468 aa, synthetic construct
IVGGWECEQHSQPWQAALYHFSTFQCGGILVHRQWVLTAAHCISDNYQLWLGRHNLFDDENTAQFVHVSESFPHPGFNMSLLENHTRQADEDYSHDLMLLRLTEPADTITDAVKVVELPTEEPEVGSTCLASGWGSIEPENFSFPDDLQCVDLKILPNDECKKAHVQKVTDFMLCVGHLEGGKDTCVGDSGGPLMCDGVLQGVTSWGYVPCGTPNKPSVAVRVLSYVKWIEDTIAENSGSSGSSGTCPPCPAPELLGGPSVFLFPPKPKDTLYITREPEVTCVVVDVSHEDPEVKFNWYVDGVEVHNAKTKPREEQYNSTYRVVSVLTVLHQDWLNGKEYKCKVSNKALPAPIEKTISKAKGQPREPQVYTLPPSRDELTKNQVSLTCLVKGFYPSDIAVEWESNGQPENNYKTTPPVLDSDGSFFLYSKLTVDKSRWQQGNVFSCSVMHEALHNHYTQKSLSLSPGK

SEQ ID NO: 63 - protein, 470 aa, synthetic construct
IVGGWECEQHSQPWQAALYHFSTFQCGGILVHRQWVLTAAHCISDNYQLWLGRHNLFDDENTAQFVHVSESFPHPGFNMSLLENHTRQADEDYSHDLMLLRLTEPADTITDAVKVVELPTEEPEVGSTCLASGWGSIEPENFSFPDDLQCVDLKILPNDECKKAHVQKVTDFMLCVGHLEGGKDTCVGDSGGPLMCDGVLQGVTSWGYVPCGTPNKPSVAVRVLSYVKWIEDTIAENSGSSGSSGGPPCPSCPAPEFLGGPSVFLFPPKPKDTLMISRTPEVTCVVVDVSQEDPEVQFNWYVDGVEVHNAKTKPREEQFNSTYRVVSVLTVLHQDWLNGKEYKCKVSNKGLPSSIEKTISKAKGQPREPQVYTLPPSQEEMTKNQVSLTCLVKGFYPSDIAVEWESNGQPENNYKTTPPVLDSDGSFFLYSRLTVDKSRWQEGNVFSCSVMHEALHNHYTQKSLSLSLGK

SEQ ID NO: 64 - protein, 470 aa, synthetic construct
IVGGWECEQHSQPWQAALYHFSTFQCGGILVHRQWVLTAAHCISDNYQLWLGRHNLFDDENTAQFVHVSESFPHPGFNMSLLENHTRQADEDYSHDLMLLRLTEPADTITDAVKVVELPTEEPEVGSTCLASGWGSIEPENFSFPDDLQCVDLKILPNDECKKAHVQKVTDFMLCVGHLEGGKDTCVGDSGGPLMCDGVLQGVTSWGYVPCGTPNKPSVAVRVLSYVKWIEDTIAENSGSSGSSGGPPCPSCPAPEFLGGPSVFLFPPKPKDTLYITREPEVTCVVVDVSQEDPEVQFNWYVDGVEVHNAKTKPREEQFNSTYRVVSVLTVLHQDWLNGKEYKCKVSNKGLPSSIEKTISKAKGQPREPQVYTLPPSQEEMTKNQVSLTCLVKGFYPSDIAVEWESNGQPENNYKTTPPVLDSDGSFFLYSRLTVDKSRWQEGNVFSCSVMHEALHNHYTQKSLSLSLGK

SEQ ID NO: 65 - protein, 471 aa, synthetic construct
IVGGWECEQHSQPWQAALYHFSTFQCGGILVHRQWVLTAAHCISDNYQLWLGRHNLFDDENTAQFVHVSESFPHPGFNMSLLENHTRQADEDYSHDLMLLRLTEPADTITDAVKVVELPTEEPEVGSTCLASGWGSIEPENFSFPDDLQCVDLKILPNDECKKAHVQKVTDFMLCVGHLEGGKDTCVGDSGGPLMCDGVLQGVTSWGYVPCGTPNKPSVAVRVLSYVKWIEDTIAENSGGGGSGGGGSTCPPCPAPELLGGPSVFLFPPKPKDTLMISRTPEVTCVVVDVSHEDPEVKFNWYVDGVEVHNAKTKPREEQYNSTYRVVSVLTVLHQDWLNGKEYKCKVSNKALPAPIEKTISKAKGQPREPQVYTLPPSRDELTKNQVSLTCLVKGFYPSDIAVEWESNGQPENNYKTTPPVLDSDGSFFLYSKLTVDKSRWQQGNVFSCSVMHEALHNHYTQKSLSLSPGK

SEQ ID NO: 66 - DNA, 1482 bp, synthetic construct
  source 1..1482: mol_type = other DNA
atgtggttcctggttctgtgcctcgccctgtccctgggggggactggtgctgcgggtggccaccatcatcatcatcatgtagatgacgatgacaagattgtgggaggctgggagtgtgagcagcattcccagccctggcaggcggctctgtaccatttcagcactttccagtgtgggggcatcctggtgcaccgccagtgggtgctcacagctgctcattgcatcagcgacaattaccagctctggctgggtcgccacaacttgtttgacgacgaaaacacagcccagtttgttcatgtcagtgagagcttcccacaccctggcttcaacatgagcctcctggagaaccacacccgccaagcagacgaggactacagccacgacctcatgctgctccgcctgacagagcctgctgataccatcacagatgctgtgaaggtcgtggagttgcccaccgaggaacccgaagtggggagcacctgtttggcttccggctggggcagcatcgaaccagagaatttctcatttccagatgatctccagtgtgtggacctcaaaatcctgcctaatgatgagtgcaaaaaagcccacgtccagaaggtgacagacttcatgctgtgtgtcggacacctggaaggtggcaaagacacctgtgtgggtgattcagggggcccgctgatgtgtgatggtgtgctccaaggtgtcacatcatggggctacgtcccttgtggcacccccaataagccttctgtcgccgtcagagtgctgtcttatgtgaagtggatcgaggacaccatagcggagaactccacatgcccaccgtgcccagcacctgaactcctggggggaccgtcagtcttcctcttccccccaaaacccaaggacaccctcatgatctcccggacccctgaggtcacatgcgtggtggtggacgtgagccacgaagaccctgaggtcaagttcaactggtacgtggacggcgtggaggtgcataatgccaagacaaagccgcgggaggagcagtacaacagcacgtaccgggtggtcagcgtcctcaccgtcctgcaccaggactggctgaatggcaaggagtacaagtgcaaggtctccaacaaagccctcccagcccccatcgagaaaaccatctccaaagccaaagggcagccccgagaaccacaggtgtacaccctgcccccatcccgggatgagctgaccaagaaccaggtcagcctgacctgcctggtcaaaggcttctatcccagcgacatcgccgtggagtgggagagcaatgggcagccggagaacaactacaagaccacgcctcccgtgctggactccgacggctccttcttcctctacagcaagctcaccgtggacaagagcaggtggcagcaggggaacgtcttctcatgctccgtgatgcatgaggctctgcacaaccactacacgcagaagagcctctccctgtctccgggtaaatga

SEQ ID NO: 67 - DNA, 1503 bp, synthetic construct
  source 1..1503: mol_type = other DNA
atgtggttcctggttctgtgcctcgccctgtccctgggggggactggtgctgcgggtggccaccatcatcatcatcatgtagatgacgatgacaagattgtgggaggctgggagtgtgagcagcattcccagccctggcaggcggctctgtaccatttcagcactttccagtgtgggggcatcctggtgcaccgccagtgggtgctcacagctgctcattgcatcagcgacaattaccagctctggctgggtcgccacaacttgtttgacgacgaaaacacagcccagtttgttcatgtcagtgagagcttcccacaccctggcttcaacatgagcctcctggagaaccacacccgccaagcagacgaggactacagccacgacctcatgctgctccgcctgacagagcctgctgataccatcacagatgctgtgaaggtcgtggagttgcccaccgaggaacccgaagtggggagcacctgtttggcttccggctggggcagcatcgaaccagagaatttctcatttccagatgatctccagtgtgtggacctcaaaatcctgcctaatgatgagtgcaaaaaagcccacgtccagaaggtgacagacttcatgctgtgtgtcggacacctggaaggtggcaaagacacctgtgtgggtgattcagggggcccgctgatgtgtgatggtgtgctccaaggtgtcacatcatggggctacgtcccttgtggcacccccaataagccttctgtcgccgtcagagtgctgtcttatgtgaagtggatcgaggacaccatagcggagaactccggaggcggttcaagttctagcacatgcccaccgtgcccagcacctgaactcctggggggaccgtcagtcttcctcttccccccaaaacccaaggacaccctcatgatctcccggacccctgaggtcacatgcgtggtggtggacgtgagccacgaagaccctgaggtcaagttcaactggtacgtggacggcgtggaggtgcataatgccaagacaaagccgcgggaggagcagtacaacagcacgtaccgggtggtcagcgtcctcaccgtcctgcaccaggactggctgaatggcaaggagtacaagtgcaaggtctccaacaaagccctcccagcccccatcgagaaaaccatctccaaagccaaagggcagccccgagaaccacaggtgtacaccctgcccccatcccgggatgagctgaccaagaaccaggtcagcctgacctgcctggtcaaaggcttctatcccagcgacatcgccgtggagtgggagagcaatgggcagccggagaacaactacaagaccacgcctcccgtgctggactccgacggctccttcttcctctacagcaagctcaccgtggacaagagcaggtggcagcaggggaacgtcttctcatgctccgtgatgcatgaggctctgcacaaccactacacgcagaagagcctctccctgtctccgggtaaatga

SEQ ID NO: 68 - DNA, 1497 bp, synthetic construct
  source 1..1497: mol_type = other DNA
atgtggttcctggttctgtgcctcgccctgtccctgggggggactggtgctgcgggtggccaccatcatcatcatcatgtagatgacgatgacaagattgtgggaggctgggagtgtgagcagcattcccagccctggcaggcggctctgtaccatttcagcactttccagtgtgggggcatcctggtgcaccgccagtgggtgctcacagctgctcattgcatcagcgacaattaccagctctggctgggtcgccacaacttgtttgacgacgaaaacacagcccagtttgttcatgtcagtgagagcttcccacaccctggcttcaacatgagcctcctggagaaccacacccgccaagcagacgaggactacagccacgacctcatgctgctccgcctgacagagcctgctgataccatcacagatgctgtgaaggtcgtggagttgcccaccgaggaacccgaagtggggagcacctgtttggcttccggctggggcagcatcgaaccagagaatttctcatttccagatgatctccagtgtgtggacctcaaaatcctgcctaatgatgagtgcaaaaaagcccacgtccagaaggtgacagacttcatgctgtgtgtcggacacctggaaggtggcaaagacacctgtgtgggtgattcagggggcccgctgatgtgtgatggtgtgctccaaggtgtcacatcatggggctacgtcccttgtggcacccccaataagccttctgtcgccgtcagagtgctgtcttatgtgaagtggatcgaggacaccatagcggagaactccgaggcagcggctaagacatgcccaccgtgcccagcacctgaactcctggggggaccgtcagtcttcctcttccccccaaaacccaaggacaccctcatgatctcccggacccctgaggtcacatgcgtggtggtggacgtgagccacgaagaccctgaggtcaagttcaactggtacgtggacggcgtggaggtgcataatgccaagacaaagccgcgggaggagcagtacaacagcacgtaccgggtggtcagcgtcctcaccgtcctgcaccaggactggctgaatggcaaggagtacaagtgcaaggtctccaacaaagccctcccagcccccatcgagaaaaccatctccaaagccaaagggcagccccgagaaccacaggtgtacaccctgcccccatcccgggatgagctgaccaagaaccaggtcagcctgacctgcctggtcaaaggcttctatcccagcgacatcgccgtggagtgggagagcaatgggcagccggagaacaactacaagaccacgcctcccgtgctggactccgacggctccttcttcctctacagcaagctcaccgtggacaagagcaggtggcagcaggggaacgtcttctcatgctccgtgatgcatgaggctctgcacaaccactacacgcagaagagcctctccctgtctccgggtaaatga

SEQ ID NO: 69 - DNA, 1509 bp, synthetic construct
  source 1..1509: mol_type = other DNA
atgtacaggatgcaactcctgtcttgcattgcactaagtcttgcacttgtcacaaacagtggtggccaccatcatcatcatcatgtagatgacgatgacaagattgtgggaggctgggagtgtgagcagcattcccagccctggcaggcggctctgtaccatttcagcactttccagtgtgggggcatcctggtgcaccgccagtgggtgctcacagctgctcattgcatcagcgacaattaccagctctggctgggtcgccacaacttgtttgacgacgaaaacacagcccagtttgttcatgtcagtgagagcttcccacaccctggcttcaacatgagcctcctggagaaccacacccgccaagcagacgaggactacagccacgacctcatgctgctccgcctgacagagcctgctgataccatcacagatgctgtgaaggtcgtggagttgcccaccgaggaacccgaagtggggagcacctgtttggcttccggctggggcagcatcgaaccagagaatttctcatttccagatgatctccagtgtgtggacctcaaaatcctgcctaatgatgagtgcaaaaaagcccacgtccagaaggtgacagacttcatgctgtgtgtcggacacctggaaggtggcaaagacacctgtgtgggtgattcagggggcccgctgatgtgtgatggtgtgctccaaggtgtcacatcatggggctacgtcccttgtggcacccccaataagccttctgtcgccgtcagagtgctgtcttatgtgaagtggatcgaggacaccatagcggagaactccggaggcggttcaagttctagcacatgcccaccgtgcccagcacctgaactcctggggggaccgtcagtcttcctcttccccccaaaacccaaggacaccctcatgatctcccggacccctgaggtcacatgcgtggtggtggacgtgagccacgaagaccctgaggtcaagttcaactggtacgtggacggcgtggaggtgcataatgccaagacaaagccgcgggaggagcagtacaacagcacgtaccgggtggtcagcgtcctcaccgtcctgcaccaggactggctgaatggcaaggagtacaagtgcaaggtctccaacaaagccctcccagcccccatcgagaaaaccatctccaaagccaaagggcagccccgagaaccacaggtgtacaccctgcccccatcccgggatgagctgaccaagaaccaggtcagcctgacctgcctggtcaaaggcttctatcccagcgacatcgccgtggagtgggagagcaatgggcagccggagaacaactacaagaccacgcctcccgtgctggactccgacggctccttcttcctctacagcaagctcaccgtggacaagagcaggtggcagcaggggaacgtcttctcatgctccgtgatgcatgaggctctgcacaaccactacacgcagaagagcctctccctgtctccgggtaaatga

SEQ ID NO: 70 - DNA, 1503 bp, synthetic construct
  source 1..1503: mol_type = other DNA
atgtacaggatgcaactcctgtcttgcattgcactaagtcttgcacttgtcacaaacagtggtggccaccatcatcatcatcatgtagatgacgatgacaagattgtgggaggctgggagtgtgagcagcattcccagccctggcaggcggctctgtaccatttcagcactttccagtgtgggggcatcctggtgcaccgccagtgggtgctcacagctgctcattgcatcagcgacaattaccagctctggctgggtcgccacaacttgtttgacgacgaaaacacagcccagtttgttcatgtcagtgagagcttcccacaccctggcttcaacatgagcctcctggagaaccacacccgccaagcagacgaggactacagccacgacctcatgctgctccgcctgacagagcctgctgataccatcacagatgctgtgaaggtcgtggagttgcccaccgaggaacccgaagtggggagcacctgtttggcttccggctggggcagcatcgaaccagagaatttctcatttccagatgatctccagtgtgtggacctcaaaatcctgcctaatgatgagtgcaaaaaagcccacgtccagaaggtgacagacttcatgctgtgtgtcggacacctggaaggtggcaaagacacctgtgtgggtgattcagggggcccgctgatgtgtgatggtgtgctccaaggtgtcacatcatggggctacgtcccttgtggcacccccaataagccttctgtcgccgtcagagtgctgtcttatgtgaagtggatcgaggacaccatagcggagaactccgaggcagcggctaagacatgcccaccgtgcccagcacctgaactcctggggggaccgtcagtcttcctcttccccccaaaacccaaggacaccctcatgatctcccggacccctgaggtcacatgcgtggtggtggacgtgagccacgaagaccctgaggtcaagttcaactggtacgtggacggcgtggaggtgcataatgccaagacaaagccgcgggaggagcagtacaacagcacgtaccgggtggtcagcgtcctcaccgtcctgcaccaggactggctgaatggcaaggagtacaagtgcaaggtctccaacaaagccctcccagcccccatcgagaaaaccatctccaaagccaaagggcagccccgagaaccacaggtgtacaccctgcccccatcccgggatgagctgaccaagaaccaggtcagcctgacctgcctggtcaaaggcttctatcccagcgacatcgccgtggagtgggagagcaatgggcagccggagaacaactacaagaccacgcctcccgtgctggactccgacggctccttcttcctctacagcaagctcaccgtggacaagagcaggtggcagcaggggaacgtcttctcatgctccgtgatgcatgaggctctgcacaaccactacacgcagaagagcctctccctgtctccgggtaaatga

SEQ ID NO: 71 - DNA, 1503 bp, synthetic construct
  source 1..1503: mol_type = other DNA
atgtggttcctggttctgtgcctcgccctgtccctgggggggactggtgctgcgggtggccaccatcatcatcatcatgtagatgacgatgacaagattgtgggaggctgggagtgtgagcagcattcccagccctggcaggcggctctgtaccatttcagcactttccagtgtgggggcatcctggtgcaccgccagtgggtgctcacagctgctcattgcatcagcgacaattaccagctctggctgggtcgccacaacttgtttgacgacgaaaacacagcccagtttgttcatgtcagtgagagcttcccacaccctggcttcaacatgagcctcctggagaaccacacccgccaagcagacgaggactacagccacgacctcatgctgctccgcctgacagagcctgctgataccatcacagatgctgtgaaggtcgtggagttgcccaccgaggaacccgaagtggggagcacctgtttggcttccggctggggcagcatcgaaccagagaatttctcatttccagatgatctccagtgtgtggacctcaaaatcctgcctaatgatgagtgcaaaaaagcccacgtccagaaggtgacagacttcatgctgtgtgtcggacacctggaaggtggcaaagacacctgtgtgggtgattcagggggcccgctgatgtgtgatggtgtgctccaaggtgtcacatcatggggctacgtcccttgtggcacccccaataagccttctgtcgccgtcagagtgctgtcttatgtgaagtggatcgaggacaccatagcggagaactccggatcaagtggctctagcggtacatgcccaccgtgcccagcacctgaactcctggggggaccgtcagtcttcctcttccccccaaaacccaaggacaccctcatgatctcccggacccctgaggtcacatgcgtggtggtggacgtgagccacgaagaccctgaggtcaagttcaactggtacgtggacggcgtggaggtgcataatgccaagacaaagccgcgggaggagcagtacaacagcacgtaccgggtggtcagcgtcctcaccgtcctgcaccaggactggctgaatggcaaggagtacaagtgcaaggtctccaacaaagccctcccagcccccatcgagaaaaccatctccaaagccaaagggcagccccgagaaccacaggtgtacaccctgcccccatcccgggatgagctgaccaagaaccaggtcagcctgacctgcctggtcaaaggcttctatcccagcgacatcgccgtggagtgggagagcaatgggcagccggagaacaactacaagaccacgcctcccgtgctggactccgacggctccttcttcctctacagcaagctcaccgtggacaagagcaggtggcagcaggggaacgtcttctcatgctccgtgatgcatgaggctctgcacaaccactacacgcagaagagcctctccctgtctccgggtaaatga

SEQ ID NO: 72 - DNA, 1503 bp, synthetic construct
  source 1..1503: mol_type = other DNA
atgtggttcctggttctgtgcctcgccctgtccctgggggggactggtgctgcgggtggccaccatcatcatcatcatgtagatgacgatgacaagattgtgggaggctgggagtgtgagcagcattcccagccctggcaggcggctctgtaccatttcagcactttccagtgtgggggcatcctggtgcaccgccagtgggtgctcacagctgctcattgcatcagcgacaattaccagctctggctgggtcgccacaacttgtttgacgacgaaaacacagcccagtttgttcatgtcagtgagagcttcccacaccctggcttcaacatgagcctcctggagaaccacacccgccaagcagacgaggactacagccacgacctcatgctgctccgcctgacagagcctgctgataccatcacagatgctgtgaaggtcgtggagttgcccaccgaggaacccgaagtggggagcacctgtttggcttccggctggggcagcatcgaaccagagaatttctcatttccagatgatctccagtgtgtggacctcaaaatcctgcctaatgatgagtgcaaaaaagcccacgtccagaaggtgacagacttcatgctgtgtgtcggacacctggaaggtggcaaagacacctgtgtgggtgattcagggggcccgctgatgtgtgatggtgtgctccaaggtgtcacatcatggggctacgtcccttgtggcacccccaataagccttctgtcgccgtcagagtgctgtcttatgtgaagtggatcgaggacaccatagcggagaactccggatcaagtggctctagcggtacatgcccaccgtgcccagcacctgaactcctggggggaccgtcagtcttcctcttccccccaaaacccaaggacaccctctacatcacccgggaacctgaggtcacatgcgtggtggtggacgtgagccacgaagaccctgaggtcaagttcaactggtacgtggacggcgtggaggtgcataatgccaagacaaagccgcgggaggagcagtacaacagcacgtaccgggtggtcagcgtcctcaccgtcctgcaccaggactggctgaatggcaaggagtacaagtgcaaggtctccaacaaagccctcccagcccccatcgagaaaaccatctccaaagccaaagggcagccccgagaaccacaggtgtacaccctgcccccatcccgggatgagctgaccaagaaccaggtcagcctgacctgcctggtcaaaggcttctatcccagcgacatcgccgtggagtgggagagcaatgggcagccggagaacaactacaagaccacgcctcccgtgctggactccgacggctccttcttcctctacagcaagctcaccgtggacaagagcaggtggcagcaggggaacgtcttctcatgctccgtgatgcatgaggctctgcacaaccactacacgcagaagagcctctccctgtctccgggtaaatga

SEQ ID NO: 73 - DNA, 1509 bp, synthetic construct
  source 1..1509: mol_type = other DNA
atgtggttcctggttctgtgcctcgccctgtccctgggggggactggtgctgcgggtggccaccatcatcatcatcatgtagatgacgatgacaagattgtgggaggctgggagtgtgagcagcattcccagccctggcaggcggctctgtaccatttcagcactttccagtgtgggggcatcctggtgcaccgccagtgggtgctcacagctgctcattgcatcagcgacaattaccagctctggctgggtcgccacaacttgtttgacgacgaaaacacagcccagtttgttcatgtcagtgagagcttcccacaccctggcttcaacatgagcctcctggagaaccacacccgccaagcagacgaggactacagccacgacctcatgctgctccgcctgacagagcctgctgataccatcacagatgctgtgaaggtcgtggagttgcccaccgaggaacccgaagtggggagcacctgtttggcttccggctggggcagcatcgaaccagagaatttctcatttccagatgatctccagtgtgtggacctcaaaatcctgcctaatgatgagtgcaaaaaagcccacgtccagaaggtgacagacttcatgctgtgtgtcggacacctggaaggtggcaaagacacctgtgtgggtgattcagggggcccgctgatgtgtgatggtgtgctccaaggtgtcacatcatggggctacgtcccttgtggcacccccaataagccttctgtcgccgtcagagtgctgtcttatgtgaagtggatcgaggacaccatagcggagaactccggatcaagtggctctagcggtggtcccccatgcccatcatgcccagcacctgagttcctggggggaccatcagtcttcctgttccccccaaaacccaaggacactctcatgatctcccggacccctgaggtcacgtgcgtggtggtggacgtgagccaggaagaccccgaggtccagttcaactggtacgtggatggcgtggaggtgcataatgccaagacaaagccgcgggaggagcagttcaacagcacgtaccgtgtggtcagcgtcctcaccgtcctgcaccaggactggctgaacggcaaggagtacaagtgcaaggtctccaacaaaggcctcccgtcctccatcgagaaaaccatctccaaagccaaagggcagccccgagagccacaggtgtacaccctgcccccatcccaggaggagatgaccaagaaccaggtcagcctgacctgcctggtcaaaggcttctaccccagcgacatcgccgtggagtgggagagcaatgggcagccggagaacaactacaagaccacgcctcccgtgctggactccgacggctccttcttcctctacagcaggctcaccgtggacaagagcaggtggcaggaggggaatgtcttctcatgctccgtgatgcatgaggctctgcacaaccactacacacagaagagcctctccctgtctctgggtaaatga

SEQ ID NO: 74 - DNA, 1509 bp, synthetic construct
  source 1..1509: mol_type = other DNA
atgtggttcctggttctgtgcctcgccctgtccctgggggggactggtgctgcgggtggccaccatcatcatcatcatgtagatgacgatgacaagattgtgggaggctgggagtgtgagcagcattcccagccctggcaggcggctctgtaccatttcagcactttccagtgtgggggcatcctggtgcaccgccagtgggtgctcacagctgctcattgcatcagcgacaattaccagctctggctgggtcgccacaacttgtttgacgacgaaaacacagcccagtttgttcatgtcagtgagagcttcccacaccctggcttcaacatgagcctcctggagaaccacacccgccaagcagacgaggactacagccacgacctcatgctgctccgcctgacagagcctgctgataccatcacagatgctgtgaaggtcgtggagttgcccaccgaggaacccgaagtggggagcacctgtttggcttccggctggggcagcatcgaaccagagaatttctcatttccagatgatctccagtgtgtggacctcaaaatcctgcctaatgatgagtgcaaaaaagcccacgtccagaaggtgacagacttcatgctgtgtgtcggacacctggaaggtggcaaagacacctgtgtgggtgattcagggggcccgctgatgtgtgatggtgtgctccaaggtgtcacatcatggggctacgtcccttgtggcacccccaataagccttctgtcgccgtcagagtgctgtcttatgtgaagtggatcgaggacaccatagcggagaactccggatcaagtggctctagcggtggtcccccatgcccatcatgcccagcacctgagttcctggggggaccatcagtcttcctgttccccccaaaacccaaggacactctctacatcacccgggagcctgaggtcacgtgcgtggtggtggacgtgagccaggaagaccccgaggtccagttcaactggtacgtggatggcgtggaggtgcataatgccaagacaaagccgcgggaggagcagttcaacagcacgtaccgtgtggtcagcgtcctcaccgtcctgcaccaggactggctgaacggcaaggagtacaagtgcaaggtctccaacaaaggcctcccgtcctccatcgagaaaaccatctccaaagccaaagggcagccccgagagccacaggtgtacaccctgcccccatcccaggaggagatgaccaagaaccaggtcagcctgacctgcctggtcaaaggcttctaccccagcgacatcgccgtggagtgggagagcaatgggcagccggagaacaactacaagaccacgcctcccgtgctggactccgacggctccttcttcctctacagcaggctcaccgtggacaagagcaggtggcaggaggggaatgtcttctcatgctccgtgatgcatgaggctctgcacaaccactacacacagaagagcctctccctgtctctgggtaaatga

SEQ ID NO: 75 - DNA, 1512 bp, synthetic construct
  source 1..1512: mol_type = other DNA
atgtggttcctggttctgtgcctcgccctgtccctgggggggactggtgctgcgggtggccaccatcatcatcatcatgtagatgacgatgacaagattgtgggaggctgggagtgtgagcagcattcccagccctggcaggcggctctgtaccatttcagcactttccagtgtgggggcatcctggtgcaccgccagtgggtgctcacagctgctcattgcatcagcgacaattaccagctctggctgggtcgccacaacttgtttgacgacgaaaacacagcccagtttgttcatgtcagtgagagcttcccacaccctggcttcaacatgagcctcctggagaaccacacccgccaagcagacgaggactacagccacgacctcatgctgctccgcctgacagagcctgctgataccatcacagatgctgtgaaggtcgtggagttgcccaccgaggaacccgaagtggggagcacctgtttggcttccggctggggcagcatcgaaccagagaatttctcatttccagatgatctccagtgtgtggacctcaaaatcctgcctaatgatgagtgcaaaaaagcccacgtccagaaggtgacagacttcatgctgtgtgtcggacacctggaaggtggcaaagacacctgtgtgggtgattcagggggcccgctgatgtgtgatggtgtgctccaaggtgtcacatcatggggctacgtcccttgtggcacccccaataagccttctgtcgccgtcagagtgctgtcttatgtgaagtggatcgaggacaccatagcggagaactccggaggcggtggatcaggaggcggtggatcaacatgcccaccgtgcccagcacctgaactcctggggggaccgtcagtcttcctcttccccccaaaacccaaggacaccctcatgatctcccggacccctgaggtcacatgcgtggtggtggacgtgagccacgaagaccctgaggtcaagttcaactggtacgtggacggcgtggaggtgcataatgccaagacaaagccgcgggaggagcagtacaacagcacgtaccgggtggtcagcgtcctcaccgtcctgcaccaggactggctgaatggcaaggagtacaagtgcaaggtctccaacaaagccctcccagcccccatcgagaaaaccatctccaaagccaaagggcagccccgagaaccacaggtgtacaccctgcccccatcccgggatgagctgaccaagaaccaggtcagcctgacctgcctggtcaaaggcttctatcccagcgacatcgccgtggagtgggagagcaatgggcagccggagaacaactacaagaccacgcctcccgtgctggactccgacggctccttcttcctctacagcaagctcaccgtggacaagagcaggtggcagcaggggaacgtcttctcatgctccgtgatgcatgaggctctgcacaaccactacacgcagaagagcctctccctgtctccgggtaaatga

SEQ ID NO: 76 - DNA, 18 bp, synthetic construct
  source 1..18: mol_type = other DNA
gtagatgacgatgacaag

SEQ ID NO: 77 - DNA, 717 bp, synthetic construct
  source 1..717: mol_type = other DNA
attgtgggaggctgggagtgtgagcagcattcccagccctggcaggcggctctgtaccatttcagcactttccagtgtgggggcatcctggtgcaccgccagtgggtgctcacagctgctcattgcatcagcgacaattaccagctctggctgggtcgccacaacttgtttgacgacgaaaacacagcccagtttgttcatgtcagtgagagcttcccacaccctggcttcaacatgagcctcctggagaaccacacccgccaagcagacgaggactacagccacgacctcatgctgctccgcctgacagagcctgctgataccatcacagatgctgtgaaggtcgtggagttgcccaccgaggaacccgaagtggggagcacctgtttggcttccggctggggcagcatcgaaccagagaatttctcatttccagatgatctccagtgtgtggacctcaaaatcctgcctaatgatgagtgcaaaaaagcccacgtccagaaggtgacagacttcatgctgtgtgtcggacacctggaaggtggcaaagacacctgtgtgggtgattcagggggcccgctgatgtgtgatggtgtgctccaaggtgtcacatcatggggctacgtcccttgtggcacccccaataagccttctgtcgccgtcagagtgctgtcttatgtgaagtggatcgaggacaccatagcggagaactcctga

SEQ ID NO: 78 - DNA, 672 bp, synthetic construct
  source 1..672: mol_type = other DNA
acatgcccaccgtgcccagcacctgaactcctggggggaccgtcagtcttcctcttccccccaaaacccaaggacaccctcatgatctcccggacccctgaggtcacatgcgtggtggtggacgtgagccacgaagaccctgaggtcaagttcaactggtacgtggacggcgtggaggtgcataatgccaagacaaagccgcgggaggagcagtacaacagcacgtaccgggtggtcagcgtcctcaccgtcctgcaccaggactggctgaatggcaaggagtacaagtgcaaggtctccaacaaagccctcccagcccccatcgagaaaaccatctccaaagccaaagggcagccccgagaaccacaggtgtacaccctgcccccatcccgggatgagctgaccaagaaccaggtcagcctgacctgcctggtcaaaggcttctatcccagcgacatcgccgtggagtgggagagcaatgggcagccggagaacaactacaagaccacgcctcccgtgctggactccgacggctccttcttcctctacagcaagctcaccgtggacaagagcaggtggcagcaggggaacgtcttctcatgctccgtgatgcatgaggctctgcacaaccactacacgcagaagagcctctccctgtctccgggtaaatga

SEQ ID NO: 79 - DNA, 678 bp, synthetic construct
  source 1..678: mol_type = other DNA
ggtcccccatgcccatcatgcccagcacctgagttcctggggggaccatcagtcttcctgttccccccaaaacccaaggacactctcatgatctcccggacccctgaggtcacgtgcgtggtggtggacgtgagccaggaagaccccgaggtccagttcaactggtacgtggatggcgtggaggtgcataatgccaagacaaagccgcgggaggagcagttcaacagcacgtaccgtgtggtcagcgtcctcaccgtcctgcaccaggactggctgaacggcaaggagtacaagtgcaaggtctccaacaaaggcctcccgtcctccatcgagaaaaccatctccaaagccaaagggcagccccgagagccacaggtgtacaccctgcccccatcccaggaggagatgaccaagaaccaggtcagcctgacctgcctggtcaaaggcttctaccccagcgacatcgccgtggagtgggagagcaatgggcagccggagaacaactacaagaccacgcctcccgtgctggactccgacggctccttcttcctctacagcaggctcaccgtggacaagagcaggtggcaggaggggaatgtcttctcatgctccgtgatgcatgaggctctgcacaaccactacacacagaagagcctctccctgtctctgggtaaatga

SEQ ID NO: 80 - DNA, 672 bp, synthetic construct
  source 1..672: mol_type = other DNA
acatgcccaccgtgcccagcacctgaactcctggggggaccgtcagtcttcctcttccccccaaaacccaaggacaccctctacatcacccgggaacctgaggtcacatgcgtggtggtggacgtgagccacgaagaccctgaggtcaagttcaactggtacgtggacggcgtggaggtgcataatgccaagacaaagccgcgggaggagcagtacaacagcacgtaccgggtggtcagcgtcctcaccgtcctgcaccaggactggctgaatggcaaggagtacaagtgcaaggtctccaacaaagccctcccagcccccatcgagaaaaccatctccaaagccaaagggcagccccgagaaccacaggtgtacaccctgcccccatcccgggatgagctgaccaagaaccaggtcagcctgacctgcctggtcaaaggcttctatcccagcgacatcgccgtggagtgggagagcaatgggcagccggagaacaactacaagaccacgcctcccgtgctggactccgacggctccttcttcctctacagcaagctcaccgtggacaagagcaggtggcagcaggggaacgtcttctcatgctccgtgatgcatgaggctctgcacaaccactacacgcagaagagcctctccctgtctccgggtaaatga

SEQ ID NO: 81 - DNA, 678 bp, synthetic construct
  source 1..678: mol_type = other DNA
ggtcccccatgcccatcatgcccagcacctgagttcctggggggaccatcagtcttcctgttccccccaaaacccaaggacactctctacatcacccgggagcctgaggtcacgtgcgtggtggtggacgtgagccaggaagaccccgaggtccagttcaactggtacgtggatggcgtggaggtgcataatgccaagacaaagccgcgggaggagcagttcaacagcacgtaccgtgtggtcagcgtcctcaccgtcctgcaccaggactggctgaacggcaaggagtacaagtgcaaggtctccaacaaaggcctcccgtcctccatcgagaaaaccatctccaaagccaaagggcagccccgagagccacaggtgtacaccctgcccccatcccaggaggagatgaccaagaaccaggtcagcctgacctgcctggtcaaaggcttctaccccagcgacatcgccgtggagtgggagagcaatgggcagccggagaacaactacaagaccacgcctcccgtgctggactccgacggctccttcttcctctacagcaggctcaccgtggacaagagcaggtggcaggaggggaatgtcttctcatgctccgtgatgcatgaggctctgcacaaccactacacacagaagagcctctccctgtctctgggtaaatga

SEQ ID NO: 82 - DNA, 18 bp, synthetic construct
  source 1..18: mol_type = other DNA
caccatcatcatcatcat

SEQ ID NO: 83 - DNA, 15 bp, synthetic construct
  source 1..15: mol_type = other DNA
ggaggcggtggatca

SEQ ID NO: 84 - DNA, 21 bp, synthetic construct
  source 1..21: mol_type = other DNA
ggatcaagtggctctagcggt

SEQ ID NO: 85 - DNA, 21 bp, synthetic construct
  source 1..21: mol_type = other DNA
ggaggcggttcaagttctagc

SEQ ID NO: 86 - DNA, 15 bp, synthetic construct
  source 1..15: mol_type = other DNA
gaggcagcggctaag

SEQ ID NO: 87 - DNA, 54 bp, synthetic construct
  source 1..54: mol_type = other DNA
atgtggttcctggttctgtgcctcgccctgtccctgggggggactggtgctgcg

SEQ ID NO: 88 - DNA, 60 bp, synthetic construct
  source 1..60: mol_type = other DNA
atgtacaggatgcaactcctgtcttgcattgcactaagtcttgcacttgtcacaaacagt

SEQ ID NO: 89 - protein, 490 aa, synthetic construct
MWFLVLCLALSLGGTGAAPPIQSRIVGGWECEQHSQPWQAALYHFSTFQCGGILVHRQWVLTAAHCISDNYQLWLGRHNLFDDENTAQFVHVSESFPHPGFNMSLLENHTRQADEDYSHDLMLLRLTEPADTITDAVKVVELPTEEPEVGSTCLASGWGSIEPENFSFPDDLQCVDLKILPNDECKKAHVQKVTDFMLCVGHLEGGKDTCVGDSGGPLMCDGVLQGVTSWGYVPCGTPNKPSVAVRVLSYVKWIEDTIAENSEAAAKTCPPCPAPELLGGPSVFLFPPKPKDTLMISRTPEVTCVVVDVSHEDPEVKFNWYVDGVEVHNAKTKPREEQYNSTYRVVSVLTVLHQDWLNGKEYKCKVSNKALPAPIEKTISKAKGQPREPQVYTLPPSRDELTKNQVSLTCLVKGFYPSDIAVEWESNGQPENNYKTTPPVLDSDGSFFLYSKLTVDKSRWQQGNVFSCSVMHEALHNHYTQKSLSLSPGK

SEQ ID NO: 90 - DNA, 1500 bp, synthetic construct
  source 1..1500: mol_type = other DNA
atgtggttcctggttctgtgcctcgccctgtccctgggggggactggtgctgcgcccccgattcagtcccgggtagatgacgatgacaagattgtgggaggctgggagtgtgagcagcattcccagccctggcaggcggctctgtaccatttcagcactttccagtgtgggggcatcctggtgcaccgccagtgggtgctcacagctgctcattgcatcagcgacaattaccagctctggctgggtcgccacaacttgtttgacgacgaaaacacagcccagtttgttcatgtcagtgagagcttcccacaccctggcttcaacatgagcctcctggagaaccacacccgccaagcagacgaggactacagccacgacctcatgctgctccgcctgacagagcctgctgataccatcacagatgctgtgaaggtcgtggagttgcccaccgaggaacccgaagtggggagcacctgtttggcttccggctggggcagcatcgaaccagagaatttctcatttccagatgatctccagtgtgtggacctcaaaatcctgcctaatgatgagtgcaaaaaagcccacgtccagaaggtgacagacttcatgctgtgtgtcggacacctggaaggtggcaaagacacctgtgtgggtgattcagggggcccgctgatgtgtgatggtgtgctccaaggtgtcacatcatggggctacgtcccttgtggcacccccaataagccttctgtcgccgtcagagtgctgtcttatgtgaagtggatcgaggacaccatagcggagaactccgaggcagcggctaagacatgcccaccgtgcccagcacctgaactcctggggggaccgtcagtcttcctcttccccccaaaacccaaggacaccctcatgatctcccggacccctgaggtcacatgcgtggtggtggacgtgagccacgaagaccctgaggtcaagttcaactggtacgtggacggcgtggaggtgcataatgccaagacaaagccgcgggaggagcagtacaacagcacgtaccgggtggtcagcgtcctcaccgtcctgcaccaggactggctgaatggcaaggagtacaagtgcaaggtctccaacaaagccctcccagcccccatcgagaaaaccatctccaaagccaaagggcagccccgagaaccacaggtgtacaccctgcccccatcccgggatgagctgaccaagaaccaggtcagcctgacctgcctggtcaaaggcttctatcccagcgacatcgccgtggagtgggagagcaatgggcagccggagaacaactacaagaccacgcctcccgtgctggactccgacggctccttcttcctctacagcaagctcaccgtggacaagagcaggtggcagcaggggaacgtcttctcatgctccgtgatgcatgaggctctgcacaaccactacacgcagaagagcctctccctgtctccgggtaaatgactcgagtgc

SEQ ID NO: 91 - protein, 268 aa, synthetic construct
MWFLVLCLALSLGGTGAAPPIQSRVDDDDKIVGGWECEQHSQPWQAALYHFSTFQCGGILVHRQWVLTAAHCISDNYQLWLGRHNLFDDENTAQFVHVSESFPHPGFNMSLLENHTRQADEDYSHDLMLLRLTEPADTITDAVKVVELPTEEPEVGSTCLASGWGSIEPENFSFPDDLQCVDLKILPNDECKKAHVQKVTDFMLCVGHLEGGKDTCVGDSGGPLMCDGVLQGVTSWGYVPCGTPNKPSVAVRVLSYVKWIEDTIAENS

SEQ ID NO: 92 - protein, 496 aa, synthetic construct
MWFLVLCLALSLGGTGAAPPIQSRVDDDDKIVGGWECEQHSQPWQAALYHFSTFQCGGILVHRQWVLTAAHCISDNYQLWLGRHNLFDDENTAQFVHVSESFPHPGFNMSLLENHTRQADEDYSHDLMLLRLTEPADTITDAVKVVELPTEEPEVGSTCLASGWGSIEPENFSFPDDLQCVDLKILPNDECKKAHVQKVTDFMLCVGHLEGGKDTCVGDSGGPLMCDGVLQGVTSWGYVPCGTPNKPSVAVRVLSYVKWIEDTIAENSEAAAKTCPPCPAPELLGGPSVFLFPPKPKDTLMISRTPEVTCVVVDVSHEDPEVKFNWYVDGVEVHNAKTKPREEQYNSTYRVVSVLTVLHQDWLNGKEYKCKVSNKALPAPIEKTISKAKGQPREPQVYTLPPSRDELTKNQVSLTCLVKGFYPSDIAVEWESNGQPENNYKTTPPVLDSDGSFFLYSKLTVDKSRWQQGNVFSCSVMHEALHNHYTQKSLSLSPGK

SEQ ID NO: 93 - protein, 472 aa, synthetic construct
PPIQSRIVGGWECEQHSQPWQAALYHFSTFQCGGILVHRQWVLTAAHCISDNYQLWLGRHNLFDDENTAQFVHVSESFPHPGFNMSLLENHTRQADEDYSHDLMLLRLTEPADTITDAVKVVELPTEEPEVGSTCLASGWGSIEPENFSFPDDLQCVDLKILPNDECKKAHVQKVTDFMLCVGHLEGGKDTCVGDSGGPLMCDGVLQGVTSWGYVPCGTPNKPSVAVRVLSYVKWIEDTIAENSEAAAKTCPPCPAPELLGGPSVFLFPPKPKDTLMISRTPEVTCVVVDVSHEDPEVKFNWYVDGVEVHNAKTKPREEQYNSTYRVVSVLTVLHQDWLNGKEYKCKVSNKALPAPIEKTISKAKGQPREPQVYTLPPSRDELTKNQVSLTCLVKGFYPSDIAVEWESNGQPENNYKTTPPVLDSDGSFFLYSKLTVDKSRWQQGNVFSCSVMHEALHNHYTQKSLSLSPGK

SEQ ID NO: 94 - protein, 244 aa, synthetic construct
PPIQSRIVGGWECEQHSQPWQAALYHFSTFQCGGILVHRQWVLTAAHCISDNYQLWLGRHNLFDDENTAQFVHVSESFPHPGFNMSLLENHTRQADEDYSHDLMLLRLTEPADTITDAVKVVELPTEEPEVGSTCLASGWGSIEPENFSFPDDLQCVDLKILPNDECKKAHVQKVTDFMLCVGHLEGGKDTCVGDSGGPLMCDGVLQGVTSWGYVPCGTPNKPSVAVRVLSYVKWIEDTIAENS

SEQ ID NO: 95 - protein, 250 aa, synthetic construct
PPIQSRVDDDDKIVGGWECEQHSQPWQAALYHFSTFQCGGILVHRQWVLTAAHCISDNYQLWLGRHNLFDDENTAQFVHVSESFPHPGFNMSLLENHTRQADEDYSHDLMLLRLTEPADTITDAVKVVELPTEEPEVGSTCLASGWGSIEPENFSFPDDLQCVDLKILPNDECKKAHVQKVTDFMLCVGHLEGGKDTCVGDSGGPLMCDGVLQGVTSWGYVPCGTPNKPSVAVRVLSYVKWIEDTIAENS

SEQ ID NO: 96 - protein, 478 aa, synthetic construct
PPIQSRVDDDDKIVGGWECEQHSQPWQAALYHFSTFQCGGILVHRQWVLTAAHCISDNYQLWLGRHNLFDDENTAQFVHVSESFPHPGFNMSLLENHTRQADEDYSHDLMLLRLTEPADTITDAVKVVELPTEEPEVGSTCLASGWGSIEPENFSFPDDLQCVDLKILPNDECKKAHVQKVTDFMLCVGHLEGGKDTCVGDSGGPLMCDGVLQGVTSWGYVPCGTPNKPSVAVRVLSYVKWIEDTIAENSEAAAKTCPPCPAPELLGGPSVFLFPPKPKDTLMISRTPEVTCVVVDVSHEDPEVKFNWYVDGVEVHNAKTKPREEQYNSTYRVVSVLTVLHQDWLNGKEYKCKVSNKALPAPIEKTISKAKGQPREPQVYTLPPSRDELTKNQVSLTCLVKGFYPSDIAVEWESNGQPENNYKTTPPVLDSDGSFFLYSKLTVDKSRWQQGNVFSCSVMHEALHNHYTQKSLSLSPGK

SEQ ID NO: 97 - DNA, 1482 bp, synthetic construct
  source 1..1482: mol_type = other DNA
atgtggttcctggttctgtgcctcgccctgtccctgggggggactggtgctgcgcccccgattcagtcccggattgtgggaggctgggagtgtgagcagcattcccagccctggcaggcggctctgtaccatttcagcactttccagtgtgggggcatcctggtgcaccgccagtgggtgctcacagctgctcattgcatcagcgacaattaccagctctggctgggtcgccacaacttgtttgacgacgaaaacacagcccagtttgttcatgtcagtgagagcttcccacaccctggcttcaacatgagcctcctggagaaccacacccgccaagcagacgaggactacagccacgacctcatgctgctccgcctgacagagcctgctgataccatcacagatgctgtgaaggtcgtggagttgcccaccgaggaacccgaagtggggagcacctgtttggcttccggctggggcagcatcgaaccagagaatttctcatttccagatgatctccagtgtgtggacctcaaaatcctgcctaatgatgagtgcaaaaaagcccacgtccagaaggtgacagacttcatgctgtgtgtcggacacctggaaggtggcaaagacacctgtgtgggtgattcagggggcccgctgatgtgtgatggtgtgctccaaggtgtcacatcatggggctacgtcccttgtggcacccccaataagccttctgtcgccgtcagagtgctgtcttatgtgaagtggatcgaggacaccatagcggagaactccgaggcagcggctaagacatgcccaccgtgcccagcacctgaactcctggggggaccgtcagtcttcctcttccccccaaaacccaaggacaccctcatgatctcccggacccctgaggtcacatgcgtggtggtggacgtgagccacgaagaccctgaggtcaagttcaactggtacgtggacggcgtggaggtgcataatgccaagacaaagccgcgggaggagcagtacaacagcacgtaccgggtggtcagcgtcctcaccgtcctgcaccaggactggctgaatggcaaggagtacaagtgcaaggtctccaacaaagccctcccagcccccatcgagaaaaccatctccaaagccaaagggcagccccgagaaccacaggtgtacaccctgcccccatcccgggatgagctgaccaagaaccaggtcagcctgacctgcctggtcaaaggcttctatcccagcgacatcgccgtggagtgggagagcaatgggcagccggagaacaactacaagaccacgcctcccgtgctggactccgacggctccttcttcctctacagcaagctcaccgtggacaagagcaggtggcagcaggggaacgtcttctcatgctccgtgatgcatgaggctctgcacaaccactacacgcagaagagcctctccctgtctccgggtaaatgactcgagtgc

SEQ ID NO: 98 - DNA, 789 bp, synthetic construct
  source 1..789: mol_type = other DNA
atgtggttcctggttctgtgcctcgccctgtccctgggggggactggtgctgcgcccccgattcagtcccggattgtgggaggctgggagtgtgagcagcattcccagccctggcaggcggctctgtaccatttcagcactttccagtgtgggggcatcctggtgcaccgccagtgggtgctcacagctgctcattgcatcagcgacaattaccagctctggctgggtcgccacaacttgtttgacgacgaaaacacagcccagtttgttcatgtcagtgagagcttcccacaccctggcttcaacatgagcctcctggagaaccacacccgccaagcagacgaggactacagccacgacctcatgctgctccgcctgacagagcctgctgataccatcacagatgctgtgaaggtcgtggagttgcccaccgaggaacccgaagtggggagcacctgtttggcttccggctggggcagcatcgaaccagagaatttctcatttccagatgatctccagtgtgtggacctcaaaatcctgcctaatgatgagtgcaaaaaagcccacgtccagaaggtgacagacttcatgctgtgtgtcggacacctggaaggtggcaaagacacctgtgtgggtgattcagggggcccgctgatgtgtgatggtgtgctccaaggtgtcacatcatggggctacgtcccttgtggcacccccaataagccttctgtcgccgtcagagtgctgtcttatgtgaagtggatcgaggacaccatagcggagaactcctga

SEQ ID NO: 99 - DNA, 807 bp, synthetic construct
  source 1..807: mol_type = other DNA
atgtggttcctggttctgtgcctcgccctgtccctgggggggactggtgctgcgcccccgattcagtcccgggtagatgacgatgacaagattgtgggaggctgggagtgtgagcagcattcccagccctggcaggcggctctgtaccatttcagcactttccagtgtgggggcatcctggtgcaccgccagtgggtgctcacagctgctcattgcatcagcgacaattaccagctctggctgggtcgccacaacttgtttgacgacgaaaacacagcccagtttgttcatgtcagtgagagcttcccacaccctggcttcaacatgagcctcctggagaaccacacccgccaagcagacgaggactacagccacgacctcatgctgctccgcctgacagagcctgctgataccatcacagatgctgtgaaggtcgtggagttgcccaccgaggaacccgaagtggggagcacctgtttggcttccggctggggcagcatcgaaccagagaatttctcatttccagatgatctccagtgtgtggacctcaaaatcctgcctaatgatgagtgcaaaaaagcccacgtccagaaggtgacagacttcatgctgtgtgtcggacacctggaaggtggcaaagacacctgtgtgggtgattcagggggcccgctgatgtgtgatggtgtgctccaaggtgtcacatcatggggctacgtcccttgtggcacccccaataagccttctgtcgccgtcagagtgctgtcttatgtgaagtggatcgaggacaccatagcggagaactcctga

SEQ ID NO: 100 - protein, 475 aa, synthetic construct
GGHHHHHHVDDDDKIVGGWECEQHSQPWQAALYHFSTFQCGGILVHRQWVLTAAHCISDNYQLWLGRHNLFDDENTAQFVHVSESFPHPGFNMSLLENHTRQADEDYSHDLMLLRLTEPADTITDAVKVVELPTEEPEVGSTCLASGWGSIEPENFSFPDDLQCVDLKILPNDECKKAHVQKVTDFMLCVGHLEGGKDTCVGDSGGPLMCDGVLQGVTSWGYVPCGTPNKPSVAVRVLSYVKWIEDTIAENSTCPPCPAPELLGGPSVFLFPPKPKDTLMISRTPEVTCVVVDVSHEDPEVKFNWYVDGVEVHNAKTKPREEQYNSTYRVVSVLTVLHQDWLNGKEYKCKVSNKALPAPIEKTISKAKGQPREPQVYTLPPSRDELTKNQVSLTCLVKGFYPSDIAVEWESNGQPENNYKTTPPVLDSDGSFFLYSKLTVDKSRWQQGNVFSCSVMHEALHNHYTQKSLSLSPGK

SEQ ID NO: 101 - protein, 482 aa, synthetic construct
GGHHHHHHVDDDDKIVGGWECEQHSQPWQAALYHFSTFQCGGILVHRQWVLTAAHCISDNYQLWLGRHNLFDDENTAQFVHVSESFPHPGFNMSLLENHTRQADEDYSHDLMLLRLTEPADTITDAVKVVELPTEEPEVGSTCLASGWGSIEPENFSFPDDLQCVDLKILPNDECKKAHVQKVTDFMLCVGHLEGGKDTCVGDSGGPLMCDGVLQGVTSWGYVPCGTPNKPSVAVRVLSYVKWIEDTIAENSGGGSSSSTCPPCPAPELLGGPSVFLFPPKPKDTLMISRTPEVTCVVVDVSHEDPEVKFNWYVDGVEVHNAKTKPREEQYNSTYRVVSVLTVLHQDWLNGKEYKCKVSNKALPAPIEKTISKAKGQPREPQVYTLPPSRDELTKNQVSLTCLVKGFYPSDIAVEWESNGQPENNYKTTPPVLDSDGSFFLYSKLTVDKSRWQQGNVFSCSVMHEALHNHYTQKSLSLSPGK

SEQ ID NO: 102 - protein, 480 aa, synthetic construct
GGHHHHHHVDDDDKIVGGWECEQHSQPWQAALYHFSTFQCGGILVHRQWVLTAAHCISDNYQLWLGRHNLFDDENTAQFVHVSESFPHPGFNMSLLENHTRQADEDYSHDLMLLRLTEPADTITDAVKVVELPTEEPEVGSTCLASGWGSIEPENFSFPDDLQCVDLKILPNDECKKAHVQKVTDFMLCVGHLEGGKDTCVGDSGGPLMCDGVLQGVTSWGYVPCGTPNKPSVAVRVLSYVKWIEDTIAENSEAAAKTCPPCPAPELLGGPSVFLFPPKPKDTLMISRTPEVTCVVVDVSHEDPEVKFNWYVDGVEVHNAKTKPREEQYNSTYRVVSVLTVLHQDWLNGKEYKCKVSNKALPAPIEKTISKAKGQPREPQVYTLPPSRDELTKNQVSLTCLVKGFYPSDIAVEWESNGQPENNYKTTPPVLDSDGSFFLYSKLTVDKSRWQQGNVFSCSVMHEALHNHYTQKSLSLSPGK

SEQ ID NO: 103 - protein, 482 aa, synthetic construct; identical to SEQ ID NO: 101

SEQ ID NO: 104 - protein, 480 aa, synthetic construct; identical to SEQ ID NO: 102

SEQ ID NO: 105 - protein, 482 aa, synthetic construct
GGHHHHHHVDDDDKIVGGWECEQHSQPWQAALYHFSTFQCGGILVHRQWVLTAAHCISDNYQLWLGRHNLFDDENTAQFVHVSESFPHPGFNMSLLENHTRQADEDYSHDLMLLRLTEPADTITDAVKVVELPTEEPEVGSTCLASGWGSIEPENFSFPDDLQCVDLKILPNDECKKAHVQKVTDFMLCVGHLEGGKDTCVGDSGGPLMCDGVLQGVTSWGYVPCGTPNKPSVAVRVLSYVKWIEDTIAENSGSSGSSGTCPPCPAPELLGGPSVFLFPPKPKDTLMISRTPEVTCVVVDVSHEDPEVKFNWYVDGVEVHNAKTKPREEQYNSTYRVVSVLTVLHQDWLNGKEYKCKVSNKALPAPIEKTISKAKGQPREPQVYTLPPSRDELTKNQVSLTCLVKGFYPSDIAVEWESNGQPENNYKTTPPVLDSDGSFFLYSKLTVDKSRWQQGNVFSCSVMHEALHNHYTQKSLSLSPGK

SEQ ID NO: 106 - protein, 482 aa, synthetic construct
GGHHHHHHVDDDDKIVGGWECEQHSQPWQAALYHFSTFQCGGILVHRQWVLTAAHCISDNYQLWLGRHNLFDDENTAQFVHVSESFPHPGFNMSLLENHTRQADEDYSHDLMLLRLTEPADTITDAVKVVELPTEEPEVGSTCLASGWGSIEPENFSFPDDLQCVDLKILPNDECKKAHVQKVTDFMLCVGHLEGGKDTCVGDSGGPLMCDGVLQGVTSWGYVPCGTPNKPSVAVRVLSYVKWIEDTIAENSGSSGSSGTCPPCPAPELLGGPSVFLFPPKPKDTLYITREPEVTCVVVDVSHEDPEVKFNWYVDGVEVHNAKTKPREEQYNSTYRVVSVLTVLHQDWLNGKEYKCKVSNKALPAPIEKTISKAKGQPREPQVYTLPPSRDELTKNQVSLTCLVKGFYPSDIAVEWESNGQPENNYKTTPPVLDSDGSFFLYSKLTVDKSRWQQGNVFSCSVMHEALHNHYTQKSLSLSPGK

SEQ ID NO: 107 - protein, 484 aa, synthetic construct
GGHHHHHHVDDDDKIVGGWECEQHSQPWQAALYHFSTFQCGGILVHRQWVLTAAHCISDNYQLWLGRHNLFDDENTAQFVHVSESFPHPGFNMSLLENHTRQADEDYSHDLMLLRLTEPADTITDAVKVVELPTEEPEVGSTCLASGWGSIEPENFSFPDDLQCVDLKILPNDECKKAHVQKVTDFMLCVGHLEGGKDTCVGDSGGPLMCDGVLQGVTSWGYVPCGTPNKPSVAVRVLSYVKWIEDTIAENSGSSGSSGGPPCPSCPAPEFLGGPSVFLFPPKPKDTLMISRTPEVTCVVVDVSQEDPEVQFNWYVDGVEVHNAKTKPREEQFNSTYRVVSVLTVLHQDWLNGKEYKCKVSNKGLPSSIEKTISKAKGQPREPQVYTLPPSQEEMTKNQVSLTCLVKGFYPSDIAVEWESNGQPENNYKTTPPVLDSDGSFFLYSRLTVDKSRWQEGNVFSCSVMHEALHNHYTQKSLSLSLGK

SEQ ID NO: 108 - protein, 484 aa, synthetic construct
GGHHHHHHVDDDDKIVGGWECEQHSQPWQAALYHFSTFQCGGILVHRQWVLTAAHCISDNYQLWLGRHNLFDDENTAQFVHVSESFPHPGFNMSLLENHTRQADEDYSHDLMLLRLTEPADTITDAVKVVELPTEEPEVGSTCLASGWGSIEPENFSFPDDLQCVDLKILPNDECKKAHVQKVTDFMLCVGHLEGGKDTCVGDSGGPLMCDGVLQGVTSWGYVPCGTPNKPSVAVRVLSYVKWIEDTIAENSGSSGSSGGPPCPSCPAPEFLGGPSVFLFPPKPKDTLYITREPEVTCVVVDVSQEDPEVQFNWYVDGVEVHNAKTKPREEQFNSTYRVVSVLTVLHQDWLNGKEYKCKVSNKGLPSSIEKTISKAKGQPREPQVYTLPPSQEEMTKNQVSLTCLVKGFYPSDIAVEWESNGQPENNYKTTPPVLDSDGSFFLYSRLTVDKSRWQEGNVFSCSVMHEALHNHYTQKSLSLSLGK

SEQ ID NO: 109 - protein, 485 aa, synthetic construct
GGHHHHHHVDDDDKIVGGWECEQHSQPWQAALYHFSTFQCGGILVHRQWVLTAAHCISDNYQLWLGRHNLFDDENTAQFVHVSESFPHPGFNMSLLENHTRQADEDYSHDLMLLRLTEPADTITDAVKVVELPTEEPEVGSTCLASGWGSIEPENFSFPDDLQCVDLKILPNDECKKAHVQKVTDFMLCVGHLEGGKDTCVGDSGGPLMCDGVLQGVTSWGYVPCGTPNKPSVAVRVLSYVKWIEDTIAENSGGGGSGGGGSTCPPCPAPELLGGPSVFLFPPKPKDTLMISRTPEVTCVVVDVSHEDPEVKFNWYVDGVEVHNAKTKPREEQYNSTYRVVSVLTVLHQDWLNGKEYKCKVSNKALPAPIEKTISKAKGQPREPQVYTLPPSRDELTKNQVSLTCLVKGFYPSDIAVEWESNGQPENNYKTTPPVLDSDGSFFLYSKLTVDKSRWQQGNVFSCSVMHEALHNHYTQKSLSLSPGK

SEQ ID NO: 110 - protein, 500 aa, synthetic construct
MWFLVLCLALSLGGTGAAGGHHHHHHVDDDDKIVGGWECEQHSQPWQAALYHFSTFQCGGILVHRQWVLTAAHCISDNYQLWLGRHNLFDDENTAQFVHVSESFPHPGFNMSLLENHTRQADEDYSHDLMLLRLTEPADTITDAVKVVELPTQEPEVGSTCLASGWGSIEPENFSFPDDLQCVDLKILPNDECKKVHVQKVTDFMLCVGHLEGGKDTCVGDSGGPLMCDGVLQGVTSWGYVPCGTPNKPSVAVRVLSYVKWIEDTIAENSGSSGSSGTCPPCPAPELLGGPSVFLFPPKPKDTLMISRTPEVTCVVVDVSHEDPEVKFNWYVDGVEVHNAKTKPREEQYNSTYRVVSVLTVLHQDWLNGKEYKCKVSNKALPAPIEKTISKAKGQPREPQVYTLPPSRDELTKNQVSLTCLVKGFYPSDIAVEWESNGQPENNYKTTPPVLDSDGSFFLYSKLTVDKSRWQQGNVFSCSVMHEALHNHYTQKSLSLSPGK

SEQ ID NO: 111 - protein, 482 aa, synthetic construct
GGHHHHHHVDDDDKIVGGWECEQHSQPWQAALYHFSTFQCGGILVHRQWVLTAAHCISDNYQLWLGRHNLFDDENTAQFVHVSESFPHPGFNMSLLENHTRQADEDYSHDLMLLRLTEPADTITDAVKVVELPTQEPEVGSTCLASGWGSIEPENFSFPDDLQCVDLKILPNDECKKVHVQKVTDFMLCVGHLEGGKDTCVGDSGGPLMCDGVLQGVTSWGYVPCGTPNKPSVAVRVLSYVKWIEDTIAENSGSSGSSGTCPPCPAPELLGGPSVFLFPPKPKDTLMISRTPEVTCVVVDVSHEDPEVKFNWYVDGVEVHNAKTKPREEQYNSTYRVVSVLTVLHQDWLNGKEYKCKVSNKALPAPIEKTISKAKGQPREPQVYTLPPSRDELTKNQVSLTCLVKGFYPSDIAVEWESNGQPENNYKTTPPVLDSDGSFFLYSKLTVDKSRWQQGNVFSCSVMHEALHNHYTQKSLSLSPGK

SEQ ID NO: 112 - protein, 480 aa, synthetic construct
HHHHHHVDDDDKIVGGWECEQHSQPWQAALYHFSTFQCGGILVHRQWVLTAAHCISDNYQLWLGRHNLFDDENTAQFVHVSESFPHPGFNMSLLENHTRQADEDYSHDLMLLRLTEPADTITDAVKVVELPTQEPEVGSTCLASGWGSIEPENFSFPDDLQCVDLKILPNDECKKVHVQKVTDFMLCVGHLEGGKDTCVGDSGGPLMCDGVLQGVTSWGYVPCGTPNKPSVAVRVLSYVKWIEDTIAENSGSSGSSGTCPPCPAPELLGGPSVFLFPPKPKDTLMISRTPEVTCVVVDVSHEDPEVKFNWYVDGVEVHNAKTKPREEQYNSTYRVVSVLTVLHQDWLNGKEYKCKVSNKALPAPIEKTISKAKGQPREPQVYTLPPSRDELTKNQVSLTCLVKGFYPSDIAVEWESNGQPENNYKTTPPVLDSDGSFFLYSKLTVDKSRWQQGNVFSCSVMHEALHNHYTQKSLSLSPGK

SEQ ID NO: 113 - protein, 474 aa, synthetic construct
VDDDDKIVGGWECEQHSQPWQAALYHFSTFQCGGILVHRQWVLTAAHCISDNYQLWLGRHNLFDDENTAQFVHVSESFPHPGFNMSLLENHTRQADEDYSHDLMLLRLTEPADTITDAVKVVELPTQEPEVGSTCLASGWGSIEPENFSFPDDLQCVDLKILPNDECKKVHVQKVTDFMLCVGHLEGGKDTCVGDSGGPLMCDGVLQGVTSWGYVPCGTPNKPSVAVRVLSYVKWIEDTIAENSGSSGSSGTCPPCPAPELLGGPSVFLFPPKPKDTLMISRTPEVTCVVVDVSHEDPEVKFNWYVDGVEVHNAKTKPREEQYNSTYRVVSVLTVLHQDWLNGKEYKCKVSNKALPAPIEKTISKAKGQPREPQVYTLPPSRDELTKNQVSLTCLVKGFYPSDIAVEWESNGQPENNYKTTPPVLDSDGSFFLYSKLTVDKSRWQQGNVFSCSVMHEALHNHYTQKSLSLSPGK

SEQ ID NO: 114 - protein, 468 aa, synthetic construct
IVGGWECEQHSQPWQAALYHFSTFQCGGILVHRQWVLTAAHCISDNYQLWLGRHNLFDDENTAQFVHVSESFPHPGFNMSLLENHTRQADEDYSHDLMLLRLTEPADTITDAVKVVELPTQEPEVGSTCLASGWGSIEPENFSFPDDLQCVDLKILPNDECKKVHVQKVTDFMLCVGHLEGGKDTCVGDSGGPLMCDGVLQGVTSWGYVPCGTPNKPSVAVRVLSYVKWIEDTIAENSGSSGSSGTCPPCPAPELLGGPSVFLFPPKPKDTLMISRTPEVTCVVVDVSHEDPEVKFNWYVDGVEVHNAKTKPREEQYNSTYRVVSVLTVLHQDWLNGKEYKCKVSNKALPAPIEKTISKAKGQPREPQVYTLPPSRDELTKNQVSLTCLVKGFYPSDIAVEWESNGQPENNYKTTPPVLDSDGSFFLYSKLTVDKSRWQQGNVFSCSVMHEALHNHYTQKSLSLSPGK

SEQ ID NO: 115 - protein, 238 aa, synthetic construct
IVGGWECEQHSQPWQAALYHFSTFQCGGILVHRQWVLTAAHCISDNYQLWLGRHNLFDDENTAQFVHVSESFPHPGFNMSLLENHTRQADEDYSHDLMLLRLTEPADTITDAVKVVELPTQEPEVGSTCLASGWGSIEPENFSFPDDLQCVDLKILPNDECKKVHVQKVTDFMLCVGHLEGGKDTCVGDSGGPLMCDGVLQGVTSWGYVPCGTPNKPSVAVRVLSYVKWIEDTIAENS

SEQ ID NO: 116 - DNA, 1503 bp, synthetic construct
  source 1..1503: mol_type = other DNA
atgtggttcctggttctgtgcctcgccctgtccctgggggggactggtgctgcgggtggccaccatcatcatcatcatgtagatgacgatgacaagattgtgggaggctgggagtgtgagcagcattcccagccctggcaggcggctctgtaccatttcagcactttccagtgtgggggcatcctggtgcaccgccagtgggtgctcacagctgctcattgcatcagcgacaattaccagctctggctgggtcgccacaacttgtttgacgacgaaaacacagcccagtttgttcatgtcagtgagagcttcccacaccctggcttcaacatgagcctcctggagaaccacacccgccaagcagacgaggactacagccacgacctcatgctgctccgcctgacagagcctgctgataccatcacagatgctgtgaaggtcgtggagttgcccacccaggaacccgaagtggggagcacctgtttggcttccggctggggcagcatcgaaccagagaatttctcatttccagatgatctccagtgtgtggacctcaaaatcctgcctaatgatgagtgcaaaaaagtccacgtccagaaggtgacagacttcatgctgtgtgtcggacacctggaaggtggcaaagacacctgtgtgggtgattcagggggcccgctgatgtgtgatggtgtgctccaaggtgtcacatcatggggctacgtcccttgtggcacccccaataagccttctgtcgccgtcagagtgctgtcttatgtgaagtggatcgaggacaccatagcggagaactccggatcaagtggctctagcggtacatgcccaccgtgcccagcacctgaactcctggggggaccgtcagtcttcctcttccccccaaaacccaaggacaccctcatgatctcccggacccctgaggtcacatgcgtggtggtggacgtgagccacgaagaccctgaggtcaagttcaactggtacgtggacggcgtggaggtgcataatgccaagacaaagccgcgggaggagcagtacaacagcacgtaccgggtggtcagcgtcctcaccgtcctgcaccaggactggctgaatggcaaggagtacaagtgcaaggtctccaacaaagccctcccagcccccatcgagaaaaccatctccaaagccaaagggcagccccgagaaccacaggtgtacaccctgcccccatcccgggatgagctgaccaagaaccaggtcagcctgacctgcctggtcaaaggcttctatcccagcgacatcgccgtggagtgggagagcaatgggcagccggagaacaactacaagaccacgcctcccgtgctggactccgacggctccttcttcctctacagcaagctcaccgtggacaagagcaggtggcagcaggggaacgtcttctcatgctccgtgatgcatgaggctctgcacaaccactacacgcagaagagcctctccctgtctccgggtaaatga

SEQ ID NO: 117 - protein, 238 aa, synthetic construct [sequence omitted]

SEQ ID NO: 118 - protein, 238 aa, synthetic construct
IVGGWECEQHSQPWQAALYHFSTFQCGGILVHRQWVLTAAHCISDNYQLWLGRHNLFDDENTAQFVHVSESFPHPGFNMSLLENHTRQADEDYSHDLMLLRLTEPADTITDAVKVVELPTEEPEVGSTCLASGWGSIEPENFSFPDDLQCVDLKILPNDECEKAHVQKVTDFMLCVGHLEGGKDTCVGDSGGPLMCDGVLQGVTSWGYVPCGTPNKPSVAVRVLSYVKWIEDTIAENS

SEQ ID NO: 119 - protein, 238 aa, synthetic construct
IVGGWECEQHSQPWQAALYHFSTFQCGGILVHRQWVLTAAHCISDNYQLWLGRHNLFDDENTAQFVHVSESFPHPGFNMSLLENHTRQADEDYSHDLMLLRLTEPADTITDAVKVVELPTEEPEVGSTCLASGWGSIEPENFSFPDDLQCVDLKILPNDECKKVHVQKVTDFMLCVGHLEGGKDTCVGDSGGPLMCDGVLQGVTSWGYVPCGTPNKPSVAVRVLSYVKWIEDTIAENS

SEQ ID NO: 120 - protein, 238 aa, synthetic construct [sequence omitted]

SEQ ID NO: 121 - protein, 238 aa, synthetic construct
IVGGWECEQHSQPWQAALYHFSTFQCGGILVHRQWVLTAAHCISDNYQLWLGRHNLFDDENTAQFVHVSESFPHPGFNMSLLENHTRQADEDYSHDLMLLRLTEPADTITDAVKVVELPTEEPEVGSTCLASGWGSIEPENFSFPDDLQCVDLKILPNDECEKVHVQKVTDFMLCVGHLEGGKDTCVGDSGGPLMCDGVLQGVTSWGYVPCGTPNKPSVAVRVLSYVKWIEDTIAENS

SEQ ID NO: 122 - protein, 238 aa, synthetic construct
IVGGWECEQHSQPWQAALYHFSTFQCGGILVHRQWVLTAAHCISDNYQLWLGRHNLFDDENTAQFVHVSESFPHPGFNMSLLENHTRQADEDYSHDLMLLRLTEPADTITDAVKVVELPTQEPEVGSTCLASGWGSIEPENFSFPDDLQCVDLKILPNDECEKVHVQKVTDFMLCVGHLEGGKDTCVGDSGGPLMCDGVLQGVTSWGYVPCGTPNKPSVAVRVLSYVKWIEDTIAENS

SEQ ID NO: 123 - DNA, 714 bp, synthetic construct
  source 1..714: mol_type = other DNA
attgtgggaggctgggagtgtgagcagcattcccagccctggcaggcggctctgtaccatttcagcactttccagtgtgggggcatcctggtgcaccgccagtgggtgctcacagctgctcattgcatcagcgacaattaccagctctggctgggtcgccacaacttgtttgacgacgaaaacacagcccagtttgttcatgtcagtgagagcttcccacaccctggcttcaacatgagcctcctggagaaccacacccgccaagcagacgaggactacagccacgacctcatgctgctccgcctgacagagcctgctgataccatcacagatgctgtgaaggtcgtggagttgcccacccaggaacccgaagtggggagcacctgtttggcttccggctggggcagcatcgaaccagagaatttctcatttccagatgatctccagtgtgtggacctcaaaatcctgcctaatgatgagtgcaaaaaagtccacgtccagaaggtgacagacttcatgctgtgtgtcggacacctggaaggtggcaaagacacctgtgtgggtgattcagggggcccgctgatgtgtgatggtgtgctccaaggtgtcacatcatggggctacgtcccttgtggcacccccaataagccttctgtcgccgtcagagtgctgtcttatgtgaagtggatcgaggacaccatagcggagaactcc

SEQ ID NO: 124 - protein, 500 aa, synthetic construct
MWFLVLCLALSLGGTGAAGGHHHHHHVDDDDKIVGGWECEQHSQPWQAALYHFSTFQCGGILVHRQWVLTAAHCISDNYQLWLGRHNLFDDENTAQFVHVSESFPHPGFNMSLLENHTRQADEDYSHDLMLLRLTEPADTITDAVKVVELPTQEPEVGSTCLASGWGSIEPENFSFPDDLQCVDLKILPNDECEKVHVQKVTDFMLCVGHLEGGKDTCVGDSGGPLMCDGVLQGVTSWGYVPCGTPNKPSVAVRVLSYVKWIEDTIAENSGSSGSSGTCPPCPAPELLGGPSVFLFPPKPKDTLMISRTPEVTCVVVDVSHEDPEVKFNWYVDGVEVHNAKTKPREEQYNSTYRVVSVLTVLHQDWLNGKEYKCKVSNKALPAPIEKTISKAKGQPREPQVYTLPPSRDELTKNQVSLTCLVKGFYPSDIAVEWESNGQPENNYKTTPPVLDSDGSFFLYSKLTVDKSRWQQGNVFSCSVMHEALHNHYTQKSLSLSPGK

SEQ ID NO: 125 - protein, 482 aa, synthetic construct
GGHHHHHHVDDDDKIVGGWECEQHSQPWQAALYHFSTFQCGGILVHRQWVLTAAHCISDNYQLWLGRHNLFDDENTAQFVHVSESFPHPGFNMSLLENHTRQADEDYSHDLMLLRLTEPADTITDAVKVVELPTQEPEVGSTCLASGWGSIEPENFSFPDDLQCVDLKILPNDECEKVHVQKVTDFMLCVGHLEGGKDTCVGDSGGPLMCDGVLQGVTSWGYVPCGTPNKPSVAVRVLSYVKWIEDTIAENSGSSGSSGTCPPCPAPELLGGPSVFLFPPKPKDTLMISRTPEVTCVVVDVSHEDPEVKFNWYVDGVEVHNAKTKPREEQYNSTYRVVSVLTVLHQDWLNGKEYKCKVSNKALPAPIEKTISKAKGQPREPQVYTLPPSRDELTKNQVSLTCLVKGFYPSDIAVEWESNGQPENNYKTTPPVLDSDGSFFLYSKLTVDKSRWQQGNVFSCSVMHEALHNHYTQKSLSLSPGK

SEQ ID NO: 126 - protein, 480 aa, synthetic construct
HHHHHHVDDDDKIVGGWECEQHSQPWQAALYHFSTFQCGGILVHRQWVLTAAHCISDNYQLWLGRHNLFDDENTAQFVHVSESFPHPGFNMSLLENHTRQADEDYSHDLMLLRLTEPADTITDAVKVVELPTQEPEVGSTCLASGWGSIEPENFSFPDDLQCVDLKILPNDECEKVHVQKVTDFMLCVGHLEGGKDTCVGDSGGPLMCDGVLQGVTSWGYVPCGTPNKPSVAVRVLSYVKWIEDTIAENSGSSGSSGTCPPCPAPELLGGPSVFLFPPKPKDTLMISRTPEVTCVVVDVSHEDPEVKFNWYVDGVEVHNAKTKPREEQYNSTYRVVSVLTVLHQDWLNGKEYKCKVSNKALPAPIEKTISKAKGQPREPQVYTLPPSRDELTKNQVSLTCLVKGFYPSDIAVEWESNGQPENNYKTTPPVLDSDGSFFLYSKLTVDKSRWQQGNVFSCSVMHEALHNHYTQKSLSLSPGK

SEQ ID NO: 127 - protein, 474 aa, synthetic construct
VDDDDKIVGGWECEQHSQPWQAALYHFSTFQCGGILVHRQWVLTAAHCISDNYQLWLGRHNLFDDENTAQFVHVSESFPHPGFNMSLLENHTRQADEDYSHDLMLLRLTEPADTITDAVKVVELPTQEPEVGSTCLASGWGSIEPENFSFPDDLQCVDLKILPNDECEKVHVQKVTDFMLCVGHLEGGKDTCVGDSGGPLMCDGVLQGVTSWGYVPCGTPNKPSVAVRVLSYVKWIEDTIAENSGSSGSSGTCPPCPAPELLGGPSVFLFPPKPKDTLMISRTPEVTCVVVDVSHEDPEVKFNWYVDGVEVHNAKTKPREEQYNSTYRVVSVLTVLHQDWLNGKEYKCKVSNKALPAPIEKTISKAKGQPREPQVYTLPPSRDELTKNQVSLTCLVKGFYPSDIAVEWESNGQPENNYKTTPPVLDSDGSFFLYSKLTVDKSRWQQGNVFSCSVMHEALHNHYTQKSLSLSPGK

SEQ ID NO: 128 - protein, 468 aa, synthetic construct
IVGGWECEQHSQPWQAALYHFSTFQCGGILVHRQWVLTAAHCISDNYQLWLGRHNLFDDENTAQFVHVSESFPHPGFNMSLLENHTRQADEDYSHDLMLLRLTEPADTITDAVKVVELPTQEPEVGSTCLASGWGSIEPENFSFPDDLQCVDLKILPNDECEKVHVQKVTDFMLCVGHLEGGKDTCVGDSGGPLMCDGVLQGVTSWGYVPCGTPNKPSVAVRVLSYVKWIEDTIAENSGSSGSSGTCPPCPAPELLGGPSVFLFPPKPKDTLMISRTPEVTCVVVDVSHEDPEVKFNWYVDGVEVHNAKTKPREEQYNSTYRVVSVLTVLHQDWLNGKEYKCKVSNKALPAPIEKTISKAKGQPREPQVYTLPPSRDELTKNQVSLTCLVKGFYPSDIAVEWESNGQPENNYKTTPPVLDSDGSFFLYSKLTVDKSRWQQGNVFSCSVMHEALHNHYTQKSLSLSPGK

SEQ ID NO: 129 - DNA, 1512 bp, synthetic construct
  source 1..1512: mol_type = other DNA
atgtggttcctggttctgtgcctcgccctgtccctgggggggactggtgctgcgggtggccaccatcatcatcatcatgtagatgacgatgacaagattgtgggaggctgggagtgtgagcagcattcccagccctggcaggcggctctgtaccatttcagcactttccagtgtgggggcatcctggtgcaccgccagtgggtgctcacagctgctcattgcatcagcgacaattaccagctctggctgggtcgccacaacttgtttgacgacgaaaacacagcccagtttgttcatgtcagtgagagcttcccacaccctggcttcaacatgagcctcctggagaaccacacccgccaagcagacgaggactacagccacgacctcatgctgctccgcctgacagagcctgctgataccatcacagatgctgtgaaggtcgtggagttgcccacccaggaacccgaagtggggagcacctgtttggcttccggctggggcagcatcgaaccagagaatttctcatttccagatgatctccagtgtgtggacctcaaaatcctgcctaatgatgagtgcgaaaaagtccacgtccagaaggtgacagacttcatgctgtgtgtcggacacctggaaggtggcaaagacacctgtgtgggtgattcagggggcccgctgatgtgtgatggtgtgctccaaggtgtcacatcatggggctacgtcccttgtggcacccccaataagccttctgtcgccgtcagagtgctgtcttatgtgaagtggatcgaggacaccatagcggagaactccggatcaagtggctctagcggtacatgcccaccgtgcccagcacctgaactcctggggggaccgtcagtcttcctcttccccccaaaacccaaggacaccctcatgatctcccggacccctgaggtcacatgcgtggtggtggacgtgagccacgaagaccctgaggtcaagttcaactggtacgtggacggcgtggaggtgcataatgccaagacaaagccgcgggaggagcagtacaacagcacgtaccgggtggtcagcgtcctcaccgtcctgcaccaggactggctgaatggcaaggagtacaagtgcaaggtctccaacaaagccctcccagcccccatcgagaaaaccatctccaaagccaaagggcagccccgagaaccacaggtgtacaccctgcccccatcccgggatgagctgaccaagaaccaggtcagcctgacctgcctggtcaaaggcttctatcccagcgacatcgccgtggagtgggagagcaatgggcagccggagaacaactacaagaccacgcctcccgtgctggactccgacggctccttcttcctctacagcaagctcaccgtggacaagagcaggtggcagcaggggaacgtcttctcatgctccgtgatgcatgaggctctgcacaaccactacacgcagaagagcctctccctgtctccgggtaaatgactcgagtgc

SEQ ID NO: 130 - DNA, 714 bp, synthetic construct
  source 1..714: mol_type = other DNA
attgtgggaggctgggagtgtgagcagcattcccagccctggcaggcggctctgtaccatttcagcactttccagtgtgggggcatcctggtgcaccgccagtgggtgctcacagctgctcattgcatcagcgacaattaccagctctggctgggtcgccacaacttgtttgacgacgaaaacacagcccagtttgttcatgtcagtgagagcttcccacaccctggcttcaacatgagcctcctggagaaccacacccgccaagcagacgaggactacagccacgacctcatgctgctccgcctgacagagcctgctgataccatcacagatgctgtgaaggtcgtggagttgcccacccaggaacccgaagtggggagcacctgtttggcttccggctggggcagcatcgaaccagagaatttctcatttccagatgatctccagtgtgtggacctcaaaatcctgcctaatgatgagtgcgaaaaagtccacgtccagaaggtgacagacttcatgctgtgtgtcggacacctggaaggtggcaaagacacctgtgtgggtgattcagggggcccgctgatgtgtgatggtgtgctccaaggtgtcacatcatggggctacgtcccttgtggcacccccaataagccttctgtcgccgtcagagtgctgtcttatgtgaagtggatcgaggacaccatagcggagaactcc